European Patent Application EP 4 534 677 A1, published April 9, 2025. Title: Nucleic acid molecule, vector, recombinant cell and drug for treatment of central nervous system diseases. Applicant: ＪＣＲファーマ株式会社. The sequence listing filed with the application follows.

SEQUENCE LISTING (28 sequences)

SEQ ID NO: 1 - DNA, 395 bp, synthetic construct
  source 1..395: mol_type = other DNA
gggaatgaaagaccccacctgtaggtttggcaagctaggatcaaggtcaggaacagagaaacaggagaatatgggccaaacaggatatctgtggtaagcagttcctgccccgctcagggccaagaacagttggaacaggagaatatgggccaaacaggatatctgtggtaagcagttcctgccccgctcagggccaagaacagatggtccccagatgcggtcccgccctcagcagtttctagagaaccatcagatgtttccagggtgccccaaggacctgaaatgaccctgtgccttatttgaactaaccaatcagttcgcttctcgcttctgttcgcgcgcttctgctccccgagctctatataagcagagctggtttagtgaaccgtcagatc

SEQ ID NO: 2 - DNA, 8113 bp, synthetic construct
  source 1..8113: mol_type = other DNA
gaattctaatagtaatcaattacggggtcattagttcatagcccatatatggagttccgcgttacataacttacggtaaatggcccgcctggctgaccgcccaacgacccccgcccattgacgtcaataatgacgtatgttcccatagtaacgccaatagggactttccattgacgtcaatgggtggagtatttacggtaaactgcccacttggcagtacatcaagtgtatcatatgccaagtacgccccctattgacgtcaatgacggtaaatggcccgcctggcattatgcccagtacatgaccttatgggactttcctacttggcagtacatctacgtattagtcatcgctattaccatggtgatgcggttttggcagtacatcaatgggcgtggatagcggtttgactcacggggatttccaagtctccaccccattgacgtcaatgggagtttgttttggcaccaaaatcaacgggactttccaaaatgtcgtaacaactccgccccattgacgcaaatgggcggtaggcgtgtacggtgggaggtctatataagcagagctggtttagtgaaccgggtctctctggttagaccagatctgagcctgggagctctctggctaactagggaacccactgcttaagcctcaataaagcttgccttgagtgcttcaagtagtgtgtgcccgtctgttgtgtgactctggtaactagagatccctcagacccttttagtcagtgtggaaaatctctagcagtggcgcccgaacagggacttgaaagcgaaagggaaaccagaggagctctctcgacgcaggactcggcttgctgaagcgcgcacggcaagaggcgaggggcggcgactggtgagtacgccaaaaattttgactagcggaggctagaaggagagagatgggtgcgagagcgtcagtattaagcgggggagaattagatcgcgatgggaaaaaattcggttaaggccagggggaaagaaaaaatataaattaaaacatatagtatgggcaagcagggagctagaacgattcgcagttaatcctggcctgttagaaacatcagaaggctgtagacaaatacgccgctgatcttcagacctggaggaggagatatgagggacaattggagaagtgaattatataaatataaagtagtaaaaattgaaccattaggagtagcacccaccaaggcaaagagaagagtggtgcagagagaaaaaagagcagtgggaataggagctttgttccttgggttcttgggagcagcaggaagcactatgggcgcagcgtcaatgacgctgacggtacaggccagacaattattgtctggtatagtgcagcagcagaacaatttgctgagggctattgaggcgcaacagcatctgttgcaactcacagtctggggcatcaagcagctccaggcaagaatcctggctgtggaaagatacctaaaggatcaacagctcctggggatttggggttgctctggaaaactcatttgcaccactgctgtgccttggaatgctagttggagtaataaatctctggaacagatttggaatcacacgacctggatggagtgggacagagaaattaacaattacacaagcttaatacactccttaattgaagaatcgcaaaaccagcaagaaaagaatgaacaagaattattggaattagataaatgggcaagtttgtggaattggtttaacataacaaattggctgtggtatataaaattattcataatgatagtaggaggcttggtaggtttaagaatagtttttgctgtactttctatagtgaatagagttaggcagggatattcaccattatcgtttcagacccacctcccaaccccgaggggacccgacaggcccgaaggaatagaagaagaaggtggagagagagacagagacagatccattcgattagtgaacggatctcgacggtatcgcctttaaaagaaaaggggggattggggggtacagtgcaggggaaagaatagtagacataatagcaacagacatacaaactaaagaattacaaaaacaaattacaaaaattcaaaattttcgggtttattacagggacagcagagatccagtttatcgatttaaatacgcgtgggaatgaaagaccccacctgtaggtttggcaagctaggatcaaggtcaggaacagagaaacaggagaatatgggccaaacaggatatctgtggtaagcagttcctgccccgctcagggccaagaacagttggaacaggagaatatgggccaaacaggatatctgtggtaagcagttcctgccccgctcagggccaagaacagatggtccccagatgcggtcccgccctcagcagtttctagagaaccatcagatgtttccagggtgccccaaggacctgaaatgaccctgtgccttatttgaactaaccaatcagttcgcttctcgcttctgttcgcgcgcttctgctccccgagctctatataagcagagctggtttagtgaaccgtcagatcggatccgcggccgccaccatgcctcctccaagaaccgggcggggcctgctgtggctggggctggtcctgtcctccgtctgcgtggctctgggaagcgaaactcaggcaaacagcaccacagacgccctgaatgtgctgctgatcattgtggacgatctgcgaccttccctgggctgctacggagacaagctggtgaggtctccaaacatcgatcagctggcttcacacagcctgctgttccagaatgcctttgctcagcaggccgtgtgcgcaccatcacgggtcagcttcctgaccggcaggagacctgacactaccaggctgtacgacttcaactcatattggagagtgcatgccggcaatttcagcaccatcccacagtactttaaggagaacggatatgtgacaatgagcgtggggaaagtcttccaccccggcattagctccaatcatacagacgattccccatactcctggtcttttcccccttatcacccctctagtgagaagtacgaaaacacaaaaacttgcagggggccagacggcgagctgcatgcaaatctgctgtgccccgtggacgtgctggatgtgcccgaaggaacactgcctgataagcagtccactgagcaggccattcagctgctggaaaagatgaaaacaagtgcttcacccttctttctggcagtggggtaccacaaaccacatatccccttcagatatcccaaggagtttcagaaactgtaccctctggaaaacattactctggctcccgaccctgaggtgcctgatgggctgccacccgtcgcatataacccatggatggacatccggcagcgcgaggatgtgcaggccctgaatatctctgtcccttacggcccaattcccgtggacttccagagaaagattcggcagagttactttgccagcgtctcctatctggatactcaagtgggccgcctgctgtctgctctggacgatctgcagctggccaacagcaccatcattgctttcacatccgaccacggatgggctctgggagagcatggggaatgggcaaagtatagcaatttcgatgtggccactcacgtcccactgatcttttacgtgccaggacgaaccgcaagcctgccagaggctggggaaaaactgttcccttatctggacccatttgattctgctagtcagctgatggagcccggccgacagtctatggacctggtggaactggtcagtctgttccctacactggctggactggcaggactgcaggtgcctccaagatgccctgtgccatccttccacgtcgagctgtgccgggaaggaaagaacctgctgaaacacttcaggttcagggacctggaggaagatccttacctgccagggaatccccgggagctgatcgcctacagtcagtatccccgcccttcagacattcctcagtggaactccgacaagccatctctgaaggatatcaaaattatggggtattctatccgcactattgattaccgatataccgtgtgggtcggcttcaaccctgacgagttcctggcaaacttcagcgatatccacgccggagaactgtactttgtggactcagatccactgcaggaccacaatatgtataatgattcccaggggggcgatctgttccagctgctgatgccttgactcgagcctgcaggcgcgtctggaacaatcaacctctggattacaaaatttgtgaaagattgactggtattcttaactatgttgctccttttacgctatgtggatacgctgctttaatgcctttgtatcatgctattgcttcccgtatggctttcattttctcctccttgtataaatcctggttgctgtctctttatgaggagttgtggcccgttgtcaggcaacgtggcgtggtgtgcactgtgtttgctgacgcaacccccactggttggggcattgccaccacctgtcagctcctttccgggactttcgctttccccctccctattgccacggcggaactcatcgccgcctgccttgcccgctgctggacaggggctcggctgttgggcactgacaattccgtggtgttgtcggggaagctgacgtcctttccatggctagctcgcctgtgttgccacctggattctgcgcgggacgtccttctgctacgtcccttcggccctcaatccagcggaccttccttcccgcggcctgctgccggctctgcggcctcttccgcgtcttcgccttcgccctcagacgagtcggatctccctttgggccgcctccccgcctggaattaattctgcagtcgagacctagaaaaacatggagcaatcacaagtagcaatacagcagctaccaatgctgattgtgcctggctagaagcacaagaggaggaggaggtgggttttccagtcacacctcaggtacctttaagaccaatgacttacaaggcagctgtagatcttagccactttttaaaagaaaagaggggactggaagggctaattcactcccaacgaagacaagattctagagggacagcccccccccaaagcccccagggatgtaattacgtccctcccccgctagggggcagcagcgagccgcccggggctccgctccggtccggcgctccccccgcatccccgagccggcagcgtgcggggacagcccgggcacggggaaggtggcacgggatcgctttcctctgaacgcttctcgctgctctttgagcctgcagacacctggggggatacggggaaaaagcttctgctttttgcttgtactgggtctctctggttagaccagatctgagcctgggagctctctggctaactagggaacccactgcttaagcctcaataaagcttgccttgagtgcttcaagtagtgtgtgcccgtctgttgtgtgactctggtaactagagatccctcagacccttttagtcagtgtggaaaatctctagcagtagtagttcatgtcatcttattattcagtatttataacttgcaaagaaatgaatatcagagagtgagaggccttgacattgctagcgttttaccgtcgacctctagctagagcttggcgtaatcatggtcatagctgtttcctgtgtgaaattgttatccgctcacaattccacacaacatacgagccggaagcataaagtgtaaagcctggggtgcctaatgagtgagctaactcacattaattgcgttgcgctcactgcccgctttccagtcgggaaacctgtcgtgccagctgcattaatgaatcggccaacgcgcggggagaggcggtttgcgtattgggcgctcttccgcttcctcgctcactgactcgctgcgctcggtcgttcggctgcggcgagcggtatcagctcactcaaaggcggtaatacggttatccacagaatcaggggataacgcaggaaagaacatgtgagcaaaaggccagcaaaaggccaggaaccgtaaaaaggccgcgttgctggcgtttttccataggctccgcccccctgacgagcatcacaaaaatcgacgctcaagtcagaggtggcgaaacccgacaggactataaagataccaggcgtttccccctggaagctccctcgtgcgctctcctgttccgaccctgccgcttaccggatacctgtccgcctttctcccttcgggaagcgtggcgctttctcatagctcacgctgtaggtatctcagttcggtgtaggtcgttcgctccaagctgggctgtgtgcacgaaccccccgttcagcccgaccgctgcgccttatccggtaactatcgtcttgagtccaacccggtaagacacgacttatcgccactggcagcagccactggtaacaggattagcagagcgaggtatgtaggcggtgctacagagttcttgaagtggtggcctaactacggctacactagaagaacagtatttggtatctgcgctctgctgaagccagttaccttcggaaaaagagttggtagctcttgatccggcaaacaaaccaccgctggtagcggtggtttttttgtttgcaagcagcagattacgcgcagaaaaaaaggatctcaagaagatcctttgatcttttctacggggtctgacgctcagtggaacgaaaactcacgttaagggattttggtcatgagattatcaaaaaggatcttcacctagatccttttaaattaaaaatgaagttttaaatcaatctaaagtatatatgagtaaacttggtctgacagttaccaatgcttaatcagtgaggcacctatctcagcgatctgtctatttcgttcatccatagttgcctgactccccgtcgtgtagataactacgatacgggagggcttaccatctggccccagtgctgcaatgataccgcgagacccacgctcaccggctccagatttatcagcaataaaccagccagccggaagggccgagcgcagaagtggtcctgcaactttatccgcctccatccagtctattaattgttgccgggaagctagagtaagtagttcgccagttaatagtttgcgcaacgttgttgccattgctacaggcatcgtggtgtcacgctcgtcgtttggtatggcttcattcagctccggttcccaacgatcaaggcgagttacatgatcccccatgttgtgcaaaaaagcggttagctccttcggtcctccgatcgttgtcagaagtaagttggccgcagtgttatcactcatggttatggcagcactgcataattctcttactgtcatgccatccgtaagatgcttttctgtgactggtgagtactcaaccaagtcattctgagaatagtgtatgcggcgaccgagttgctcttgcccggcgtcaatacgggataataccgcgccacatagcagaactttaaaagtgctcatcattggaaaacgttcttcggggcgaaaactctcaaggatcttaccgctgttgagatccagttcgatgtaacccactcgtgcacccaactgatcttcagcatcttttactttcaccagcgtttctgggtgagcaaaaacaggaaggcaaaatgccgcaaaaaagggaataagggcgacacggaaatgttgaatactcatactcttcctttttcaatattattgaagcatttatcagggttattgtctcatgagcggatacatatttgaatgtatttagaaaaataaacaaataggggttccgcgcacatttccccgaaaagtgccacctgacgtcgacggatcgggagatcaacttgtttattgcagcttataatggttacaaataaagcaatagcatcacaaatttcacaaataaagcatttttttcactgcattctagttgtggtttgtccaaactcatcaatgtatcttatcatgtctggatcaactggataactcaagctaaccaaaatcatcccaaacttcccaccccataccctattaccactgccaattacctgtggtttcatttactctaaacctgtgattcctctgaattattttcattttaaagaaattgtatttgttaaatatgtactacaaacttagtagt

SEQ ID NO: 3 - DNA, 1653 bp, synthetic construct
  source 1..1653: mol_type = other DNA
atgcctcctccaagaaccgggcggggcctgctgtggctggggctggtcctgtcctccgtctgcgtggctctgggaagcgaaactcaggcaaacagcaccacagacgccctgaatgtgctgctgatcattgtggacgatctgcgaccttccctgggctgctacggagacaagctggtgaggtctccaaacatcgatcagctggcttcacacagcctgctgttccagaatgcctttgctcagcaggccgtgtgcgcaccatcacgggtcagcttcctgaccggcaggagacctgacactaccaggctgtacgacttcaactcatattggagagtgcatgccggcaatttcagcaccatcccacagtactttaaggagaacggatatgtgacaatgagcgtggggaaagtcttccaccccggcattagctccaatcatacagacgattccccatactcctggtcttttcccccttatcacccctctagtgagaagtacgaaaacacaaaaacttgcagggggccagacggcgagctgcatgcaaatctgctgtgccccgtggacgtgctggatgtgcccgaaggaacactgcctgataagcagtccactgagcaggccattcagctgctggaaaagatgaaaacaagtgcttcacccttctttctggcagtggggtaccacaaaccacatatccccttcagatatcccaaggagtttcagaaactgtaccctctggaaaacattactctggctcccgaccctgaggtgcctgatgggctgccacccgtcgcatataacccatggatggacatccggcagcgcgaggatgtgcaggccctgaatatctctgtcccttacggcccaattcccgtggacttccagagaaagattcggcagagttactttgccagcgtctcctatctggatactcaagtgggccgcctgctgtctgctctggacgatctgcagctggccaacagcaccatcattgctttcacatccgaccacggatgggctctgggagagcatggggaatgggcaaagtatagcaatttcgatgtggccactcacgtcccactgatcttttacgtgccaggacgaaccgcaagcctgccagaggctggggaaaaactgttcccttatctggacccatttgattctgctagtcagctgatggagcccggccgacagtctatggacctggtggaactggtcagtctgttccctacactggctggactggcaggactgcaggtgcctccaagatgccctgtgccatccttccacgtcgagctgtgccgggaaggaaagaacctgctgaaacacttcaggttcagggacctggaggaagatccttacctgccagggaatccccgggagctgatcgcctacagtcagtatccccgcccttcagacattcctcagtggaactccgacaagccatctctgaaggatatcaaaattatggggtattctatccgcactattgattaccgatataccgtgtgggtcggcttcaaccctgacgagttcctggcaaacttcagcgatatccacgccggagaactgtactttgtggactcagatccactgcaggaccacaatatgtataatgattcccaggggggcgatctgttccagctgctgatgccttga

SEQ ID NO: 4 - protein, 550 aa, synthetic construct
MPPPRTGRGLLWLGLVLSSVCVALGSETQANSTTDALNVLLIIVDDLRPSLGCYGDKLVRSPNIDQLASHSLLFQNAFAQQAVCAPSRVSFLTGRRPDTTRLYDFNSYWRVHAGNFSTIPQYFKENGYVTMSVGKVFHPGISSNHTDDSPYSWSFPPYHPSSEKYENTKTCRGPDGELHANLLCPVDVLDVPEGTLPDKQSTEQAIQLLEKMKTSASPFFLAVGYHKPHIPFRYPKEFQKLYPLENITLAPDPEVPDGLPPVAYNPWMDIRQREDVQALNISVPYGPIPVDFQRKIRQSYFASVSYLDTQVGRLLSALDDLQLANSTIIAFTSDHGWALGEHGEWAKYSNFDVATHVPLIFYVPGRTASLPEAGEKLFPYLDPFDSASQLMEPGRQSMDLVELVSLFPTLAGLAGLQVPPRCPVPSFHVELCREGKNLLKHFRFRDLEEDPYLPGNPRELIAYSQYPRPSDIPQWNSDKPSLKDIKIMGYSIRTIDYRYTVWVGFNPDEFLANFSDIHAGELYFVDSDPLQDHNMYNDSQGGDLFQLLMP

SEQ ID NO: 5 - DNA, 783 bp, synthetic construct
  source 1..783: mol_type = other DNA
atggaaacccccgctcagctgctgttcctgctgctgctgtggctgcccgatacaaccggcgacattcagatgactcagtcccctgcttccctgtccgcctctctggaggagatcgtgaccatcacatgccaggcctcccaggacatcggcaactggctggcctggtatcagcagaagcctggcaagtctccacagctgctgatctacggagccacctctctggcagacggagtgccaagcaggttcagcggctccagatctggcacacagttttctctgaagatcagcagggtgcaggtggaggatatcggcatctactattgcctgcaggcctataataccccatggacattcggcggaggaaccaagctggagctgaagagaggaggaggaggatccggaggaggaggatctggaggaggaggatccgaggtgcagctggtggagagcggaggaggcctggtgcagcctggcaacagcctgaccctgtcctgcgtggcctctggcttcacattttccaattacggcatgcactggatccggcaggccccaaagaagggcctggagtggatcgccatgatctactatgacagctccaagatgaactatgccgataccgtgaagggccggttcacaatcagccgcgacaactccaagaataccctgtacctggagatgaacagcctgcgctctgaggacaccgccatgtactattgtgccgtgcccacaagccactatgtggtggacgtgtggggacagggcgtgtccgtgaccgtgtctagc

SEQ ID NO: 6 - protein, 261 aa, synthetic construct
METPAQLLFLLLLWLPDTTGDIQMTQSPASLSASLEEIVTITCQASQDIGNWLAWYQQKPGKSPQLLIYGATSLADGVPSRFSGSRSGTQFSLKISRVQVEDIGIYYCLQAYNTPWTFGGGTKLELKRGGGGSGGGGSGGGGSEVQLVESGGGLVQPGNSLTLSCVASGFTFSNYGMHWIRQAPKKGLEWIAMIYYDSSKMNYADTVKGRFTISRDNSKNTLYLEMNSLRSEDTAMYYCAVPTSHYVVDVWGQGVSVTVSS

SEQ ID NO: 7 - DNA, 2406 bp, synthetic construct
  source 1..2406: mol_type = other DNA
atggaaacccccgctcagctgctgttcctgctgctgctgtggctgcccgatacaaccggcgacattcagatgactcagtcccctgcttccctgtccgcctctctggaggagatcgtgaccatcacatgccaggcctcccaggacatcggcaactggctggcctggtatcagcagaagcctggcaagtctccacagctgctgatctacggagccacctctctggcagacggagtgccaagcaggttcagcggctccagatctggcacacagttttctctgaagatcagcagggtgcaggtggaggatatcggcatctactattgcctgcaggcctataataccccatggacattcggcggaggaaccaagctggagctgaagagaggaggaggaggatccggaggaggaggatctggaggaggaggatccgaggtgcagctggtggagagcggaggaggcctggtgcagcctggcaacagcctgaccctgtcctgcgtggcctctggcttcacattttccaattacggcatgcactggatccggcaggccccaaagaagggcctggagtggatcgccatgatctactatgacagctccaagatgaactatgccgataccgtgaagggccggttcacaatcagccgcgacaactccaagaataccctgtacctggagatgaacagcctgcgctctgaggacaccgccatgtactattgtgccgtgcccacaagccactatgtggtggacgtgtggggacagggcgtgtccgtgaccgtgtctagcggaggaggaggatccggaggaggaggatctggaggaggaggatcctctgagacacaggccaacagcaccacagacgccctgaatgtgctgctgatcatcgtggacgatctgcggccctccctgggatgctacggcgacaagctggtgcgctctcctaacatcgatcagctggccagccactccctgctgttccagaatgcctttgcccagcaggccgtgtgcgcaccaagccgggtgtccttcctgaccggcaggaggcccgacaccacacggctgtacgacttcaactcttattggcgcgtgcacgccggcaatttcagcaccatccctcagtactttaaggagaacggctatgtgacaatgagcgtgggcaaggtgttccacccaggcatcagctccaatcacacagacgattccccttactcttggagctttcccccttatcacccatctagcgagaagtacgagaacaccaagacatgcaggggacctgacggagagctgcacgcaaatctgctgtgcccagtggacgtgctggatgtgccagagggcaccctgcccgataagcagagcacagagcaggccatccagctgctggagaagatgaagacctccgcctctcccttctttctggccgtgggctaccacaagccacacatccccttcagatatccaaaggagtttcagaagctgtaccccctggagaacatcacactggcaccagaccctgaggtgccagatggcctgccacccgtggcctataacccttggatggacatccggcagcgcgaggatgtgcaggccctgaatatctctgtgccttacggcccaatccccgtggacttccagcggaagatccgccagagctactttgccagcgtgtcctatctggatacccaagtgggccgcctgctgtccgccctggacgatctgcagctggccaactccaccatcatcgccttcacatctgaccacggatgggcactgggagagcacggagagtgggccaagtattctaatttcgatgtggccacccacgtgcctctgatcttttacgtgccaggaaggacagcctccctgcctgaggcaggagagaagctgttcccctacctggacccttttgattctgccagccagctgatggagccaggccgccagagcatggacctggtggagctggtgtccctgttccccaccctggcaggcctggcaggcctgcaggtgcctccaaggtgccctgtgcccagcttccacgtggagctgtgcagagagggcaagaacctgctgaagcacttcaggttcagggacctggaggaggatccttacctgccaggcaatcccagggagctgatcgcctacagccagtatcccagaccttccgacatcccccagtggaactctgacaagcctagcctgaaggatatcaagatcatgggctattccatcaggaccatcgattacagatatacagtgtgggtgggcttcaacccagacgagttcctggccaatttttctgatatccacgccggcgagctgtactttgtggacagcgatcccctgcaggaccacaatatgtataacgactcccaggggggcgatctgttccagctgctgatgccatga

SEQ ID NO: 8 - protein, 801 aa, synthetic construct
METPAQLLFLLLLWLPDTTGDIQMTQSPASLSASLEEIVTITCQASQDIGNWLAWYQQKPGKSPQLLIYGATSLADGVPSRFSGSRSGTQFSLKISRVQVEDIGIYYCLQAYNTPWTFGGGTKLELKRGGGGSGGGGSGGGGSEVQLVESGGGLVQPGNSLTLSCVASGFTFSNYGMHWIRQAPKKGLEWIAMIYYDSSKMNYADTVKGRFTISRDNSKNTLYLEMNSLRSEDTAMYYCAVPTSHYVVDVWGQGVSVTVSSGGGGSGGGGSGGGGSSETQANSTTDALNVLLIIVDDLRPSLGCYGDKLVRSPNIDQLASHSLLFQNAFAQQAVCAPSRVSFLTGRRPDTTRLYDFNSYWRVHAGNFSTIPQYFKENGYVTMSVGKVFHPGISSNHTDDSPYSWSFPPYHPSSEKYENTKTCRGPDGELHANLLCPVDVLDVPEGTLPDKQSTEQAIQLLEKMKTSASPFFLAVGYHKPHIPFRYPKEFQKLYPLENITLAPDPEVPDGLPPVAYNPWMDIRQREDVQALNISVPYGPIPVDFQRKIRQSYFASVSYLDTQVGRLLSALDDLQLANSTIIAFTSDHGWALGEHGEWAKYSNFDVATHVPLIFYVPGRTASLPEAGEKLFPYLDPFDSASQLMEPGRQSMDLVELVSLFPTLAGLAGLQVPPRCPVPSFHVELCREGKNLLKHFRFRDLEEDPYLPGNPRELIAYSQYPRPSDIPQWNSDKPSLKDIKIMGYSIRTIDYRYTVWVGFNPDEFLANFSDIHAGELYFVDSDPLQDHNMYNDSQGGDLFQLLMP

SEQ ID NO: 9 - protein, 5 aa, synthetic construct
GGGGS

SEQ ID NO: 10 - protein, 6 aa, synthetic construct
GGGGGS

SEQ ID NO: 11 - protein, 5 aa, synthetic construct
SGGGG

SEQ ID NO: 12 - DNA, 6456 bp, synthetic construct
  source 1..6456: mol_type = other DNA
gaattctaatagtaatcaattacggggtcattagttcatagcccatatatggagttccgcgttacataacttacggtaaatggcccgcctggctgaccgcccaacgacccccgcccattgacgtcaataatgacgtatgttcccatagtaacgccaatagggactttccattgacgtcaatgggtggagtatttacggtaaactgcccacttggcagtacatcaagtgtatcatatgccaagtacgccccctattgacgtcaatgacggtaaatggcccgcctggcattatgcccagtacatgaccttatgggactttcctacttggcagtacatctacgtattagtcatcgctattaccatggtgatgcggttttggcagtacatcaatgggcgtggatagcggtttgactcacggggatttccaagtctccaccccattgacgtcaatgggagtttgttttggcaccaaaatcaacgggactttccaaaatgtcgtaacaactccgccccattgacgcaaatgggcggtaggcgtgtacggtgggaggtctatataagcagagctggtttagtgaaccgggtctctctggttagaccagatctgagcctgggagctctctggctaactagggaacccactgcttaagcctcaataaagcttgccttgagtgcttcaagtagtgtgtgcccgtctgttgtgtgactctggtaactagagatccctcagacccttttagtcagtgtggaaaatctctagcagtggcgcccgaacagggacttgaaagcgaaagggaaaccagaggagctctctcgacgcaggactcggcttgctgaagcgcgcacggcaagaggcgaggggcggcgactggtgagtacgccaaaaattttgactagcggaggctagaaggagagagatgggtgcgagagcgtcagtattaagcgggggagaattagatcgcgatgggaaaaaattcggttaaggccagggggaaagaaaaaatataaattaaaacatatagtatgggcaagcagggagctagaacgattcgcagttaatcctggcctgttagaaacatcagaaggctgtagacaaatacgccgctgatcttcagacctggaggaggagatatgagggacaattggagaagtgaattatataaatataaagtagtaaaaattgaaccattaggagtagcacccaccaaggcaaagagaagagtggtgcagagagaaaaaagagcagtgggaataggagctttgttccttgggttcttgggagcagcaggaagcactatgggcgcagcgtcaatgacgctgacggtacaggccagacaattattgtctggtatagtgcagcagcagaacaatttgctgagggctattgaggcgcaacagcatctgttgcaactcacagtctggggcatcaagcagctccaggcaagaatcctggctgtggaaagatacctaaaggatcaacagctcctggggatttggggttgctctggaaaactcatttgcaccactgctgtgccttggaatgctagttggagtaataaatctctggaacagatttggaatcacacgacctggatggagtgggacagagaaattaacaattacacaagcttaatacactccttaattgaagaatcgcaaaaccagcaagaaaagaatgaacaagaattattggaattagataaatgggcaagtttgtggaattggtttaacataacaaattggctgtggtatataaaattattcataatgatagtaggaggcttggtaggtttaagaatagtttttgctgtactttctatagtgaatagagttaggcagggatattcaccattatcgtttcagacccacctcccaaccccgaggggacccgacaggcccgaaggaatagaagaagaaggtggagagagagacagagacagatccattcgattagtgaacggatctcgacggtatcgcctttaaaagaaaaggggggattggggggtacagtgcaggggaaagaatagtagacataatagcaacagacatacaaactaaagaattacaaaaacaaattacaaaaattcaaaattttcgggtttattacagggacagcagagatccagtttatcgatttaaatacgcgtgggaatgaaagaccccacctgtaggtttggcaagctaggatcaaggtcaggaacagagaaacaggagaatatgggccaaacaggatatctgtggtaagcagttcctgccccgctcagggccaagaacagttggaacaggagaatatgggccaaacaggatatctgtggtaagcagttcctgccccgctcagggccaagaacagatggtccccagatgcggtcccgccctcagcagtttctagagaaccatcagatgtttccagggtgccccaaggacctgaaatgaccctgtgccttatttgaactaaccaatcagttcgcttctcgcttctgttcgcgcgcttctgctccccgagctctatataagcagagctggtttagtgaaccgtcagatcggatccgcggccgcctcgagcctgcaggcgcgtctggaacaatcaacctctggattacaaaatttgtgaaagattgactggtattcttaactatgttgctccttttacgctatgtggatacgctgctttaatgcctttgtatcatgctattgcttcccgtatggctttcattttctcctccttgtataaatcctggttgctgtctctttatgaggagttgtggcccgttgtcaggcaacgtggcgtggtgtgcactgtgtttgctgacgcaacccccactggttggggcattgccaccacctgtcagctcctttccgggactttcgctttccccctccctattgccacggcggaactcatcgccgcctgccttgcccgctgctggacaggggctcggctgttgggcactgacaattccgtggtgttgtcggggaagctgacgtcctttccatggctagctcgcctgtgttgccacctggattctgcgcgggacgtccttctgctacgtcccttcggccctcaatccagcggaccttccttcccgcggcctgctgccggctctgcggcctcttccgcgtcttcgccttcgccctcagacgagtcggatctccctttgggccgcctccccgcctggaattaattctgcagtcgagacctagaaaaacatggagcaatcacaagtagcaatacagcagctaccaatgctgattgtgcctggctagaagcacaagaggaggaggaggtgggttttccagtcacacctcaggtacctttaagaccaatgacttacaaggcagctgtagatcttagccactttttaaaagaaaagaggggactggaagggctaattcactcccaacgaagacaagattctagagggacagcccccccccaaagcccccagggatgtaattacgtccctcccccgctagggggcagcagcgagccgcccggggctccgctccggtccggcgctccccccgcatccccgagccggcagcgtgcggggacagcccgggcacggggaaggtggcacgggatcgctttcctctgaacgcttctcgctgctctttgagcctgcagacacctggggggatacggggaaaaagcttctgctttttgcttgtactgggtctctctggttagaccagatctgagcctgggagctctctggctaactagggaacccactgcttaagcctcaataaagcttgccttgagtgcttcaagtagtgtgtgcccgtctgttgtgtgactctggtaactagagatccctcagacccttttagtcagtgtggaaaatctctagcagtagtagttcatgtcatcttattattcagtatttataacttgcaaagaaatgaatatcagagagtgagaggccttgacattgctagcgttttaccgtcgacctctagctagagcttggcgtaatcatggtcatagctgtttcctgtgtgaaattgttatccgctcacaattccacacaacatacgagccggaagcataaagtgtaaagcctggggtgcctaatgagtgagctaactcacattaattgcgttgcgctcactgcccgctttccagtcgggaaacctgtcgtgccagctgcattaatgaatcggccaacgcgcggggagaggcggtttgcgtattgggcgctcttccgcttcctcgctcactgactcgctgcgctcggtcgttcggctgcggcgagcggtatcagctcactcaaaggcggtaatacggttatccacagaatcaggggataacgcaggaaagaacatgtgagcaaaaggccagcaaaaggccaggaaccgtaaaaaggccgcgttgctggcgtttttccataggctccgcccccctgacgagcatcacaaaaatcgacgctcaagtcagaggtggcgaaacccgacaggactataaagataccaggcgtttccccctggaagctccctcgtgcgctctcctgttccgaccctgccgcttaccggatacctgtccgcctttctcccttcgggaagcgtggcgctttctcatagctcacgctgtaggtatctcagttcggtgtaggtcgttcgctccaagctgggctgtgtgcacgaaccccccgttcagcccgaccgctgcgccttatccggtaactatcgtcttgagtccaacccggtaagacacgacttatcgccactggcagcagccactggtaacaggattagcagagcgaggtatgtaggcggtgctacagagttcttgaagtggtggcctaactacggctacactagaagaacagtatttggtatctgcgctctgctgaagccagttaccttcggaaaaagagttggtagctcttgatccggcaaacaaaccaccgctggtagcggtggtttttttgtttgcaagcagcagattacgcgcagaaaaaaaggatctcaagaagatcctttgatcttttctacggggtctgacgctcagtggaacgaaaactcacgttaagggattttggtcatgagattatcaaaaaggatcttcacctagatccttttaaattaaaaatgaagttttaaatcaatctaaagtatatatgagtaaacttggtctgacagttaccaatgcttaatcagtgaggcacctatctcagcgatctgtctatttcgttcatccatagttgcctgactccccgtcgtgtagataactacgatacgggagggcttaccatctggccccagtgctgcaatgataccgcgagacccacgctcaccggctccagatttatcagcaataaaccagccagccggaagggccgagcgcagaagtggtcctgcaactttatccgcctccatccagtctattaattgttgccgggaagctagagtaagtagttcgccagttaatagtttgcgcaacgttgttgccattgctacaggcatcgtggtgtcacgctcgtcgtttggtatggcttcattcagctccggttcccaacgatcaaggcgagttacatgatcccccatgttgtgcaaaaaagcggttagctccttcggtcctccgatcgttgtcagaagtaagttggccgcagtgttatcactcatggttatggcagcactgcataattctcttactgtcatgccatccgtaagatgcttttctgtgactggtgagtactcaaccaagtcattctgagaatagtgtatgcggcgaccgagttgctcttgcccggcgtcaatacgggataataccgcgccacatagcagaactttaaaagtgctcatcattggaaaacgttcttcggggcgaaaactctcaaggatcttaccgctgttgagatccagttcgatgtaacccactcgtgcacccaactgatcttcagcatcttttactttcaccagcgtttctgggtgagcaaaaacaggaaggcaaaatgccgcaaaaaagggaataagggcgacacggaaatgttgaatactcatactcttcctttttcaatattattgaagcatttatcagggttattgtctcatgagcggatacatatttgaatgtatttagaaaaataaacaaataggggttccgcgcacatttccccgaaaagtgccacctgacgtcgacggatcgggagatcaacttgtttattgcagcttataatggttacaaataaagcaatagcatcacaaatttcacaaataaagcatttttttcactgcattctagttgtggtttgtccaaactcatcaatgtatcttatcatgtctggatcaactggataactcaagctaaccaaaatcatcccaaacttcccaccccataccctattaccactgccaattacctgtggtttcatttactctaaacctgtgattcctctgaattattttcattttaaagaaattgtatttgttaaatatgtactacaaacttagtagt

SEQ ID NO: 13 - DNA, 8922 bp, synthetic construct
  source 1..8922: mol_type = other DNA
gaattctaatagtaatcaattacggggtcattagttcatagcccatatatggagttccgcgttacataacttacggtaaatggcccgcctggctgaccgcccaacgacccccgcccattgacgtcaataatgacgtatgttcccatagtaacgccaatagggactttccattgacgtcaatgggtggagtatttacggtaaactgcccacttggcagtacatcaagtgtatcatatgccaagtacgccccctattgacgtcaatgacggtaaatggcccgcctggcattatgcccagtacatgaccttatgggactttcctacttggcagtacatctacgtattagtcatcgctattaccatggtgatgcggttttggcagtacatcaatgggcgtggatagcggtttgactcacggggatttccaagtctccaccccattgacgtcaatgggagtttgttttggcaccaaaatcaacgggactttccaaaatgtcgtaacaactccgccccattgacgcaaatgggcggtaggcgtgtacggtgggaggtctatataagcagagctggtttagtgaaccgggtctctctggttagaccagatctgagcctgggagctctctggctaactagggaacccactgcttaagcctcaataaagcttgccttgagtgcttcaagtagtgtgtgcccgtctgttgtgtgactctggtaactagagatccctcagacccttttagtcagtgtggaaaatctctagcagtggcgcccgaacagggacttgaaagcgaaagggaaaccagaggagctctctcgacgcaggactcggcttgctgaagcgcgcacggcaagaggcgaggggcggcgactggtgagtacgccaaaaattttgactagcggaggctagaaggagagagatgggtgcgagagcgtcagtattaagcgggggagaattagatcgcgatgggaaaaaattcggttaaggccagggggaaagaaaaaatataaattaaaacatatagtatgggcaagcagggagctagaacgattcgcagttaatcctggcctgttagaaacatcagaaggctgtagacaaatacgccgctgatcttcagacctggaggaggagatatgagggacaattggagaagtgaattatataaatataaagtagtaaaaattgaaccattaggagtagcacccaccaaggcaaagagaagagtggtgcagagagaaaaaagagcagtgggaataggagctttgttccttgggttcttgggagcagcaggaagcactatgggcgcagcgtcaatgacgctgacggtacaggccagacaattattgtctggtatagtgcagcagcagaacaatttgctgagggctattgaggcgcaacagcatctgttgcaactcacagtctggggcatcaagcagctccaggcaagaatcctggctgtggaaagatacctaaaggatcaacagctcctggggatttggggttgctctggaaaactcatttgcaccactgctgtgccttggaatgctagttggagtaataaatctctggaacagatttggaatcacacgacctggatggagtgggacagagaaattaacaattacacaagcttaatacactccttaattgaagaatcgcaaaaccagcaagaaaagaatgaacaagaattattggaattagataaatgggcaagtttgtggaattggtttaacataacaaattggctgtggtatataaaattattcataatgatagtaggaggcttggtaggtttaagaatagtttttgctgtactttctatagtgaatagagttaggcagggatattcaccattatcgtttcagacccacctcccaaccccgaggggacccgacaggcccgaaggaatagaagaagaaggtggagagagagacagagacagatccattcgattagtgaacggatctcgacggtatcgcctttaaaagaaaaggggggattggggggtacagtgcaggggaaagaatagtagacataatagcaacagacatacaaactaaagaattacaaaaacaaattacaaaaattcaaaattttcgggtttattacagggacagcagagatccagtttatcgatttaaatacgcgtgggaatgaaagaccccacctgtaggtttggcaagctaggatcaaggtcaggaacagagaaacaggagaatatgggccaaacaggatatctgtggtaagcagttcctgccccgctcagggccaagaacagttggaacaggagaatatgggccaaacaggatatctgtggtaagcagttcctgccccgctcagggccaagaacagatggtccccagatgcggtcccgccctcagcagtttctagagaaccatcagatgtttccagggtgccccaaggacctgaaatgaccctgtgccttatttgaactaaccaatcagttcgcttctcgcttctgttcgcgcgcttctgctccccgagctctatataagcagagctggtttagtgaaccgtcagatcggatccgcggccgctctagcccgggcggatcccccgggctgcaggaattcaccatggaaacccccgctcagctgctgttcctgctgctgctgtggctgcccgatacaaccggcgacattcagatgactcagtcccctgcttccctgtccgcctctctggaggagatcgtgaccatcacatgccaggcctcccaggacatcggcaactggctggcctggtatcagcagaagcctggcaagtctccacagctgctgatctacggagccacctctctggcagacggagtgccaagcaggttcagcggctccagatctggcacacagttttctctgaagatcagcagggtgcaggtggaggatatcggcatctactattgcctgcaggcctataataccccatggacattcggcggaggaaccaagctggagctgaagagaggaggaggaggatccggaggaggaggatctggaggaggaggatccgaggtgcagctggtggagagcggaggaggcctggtgcagcctggcaacagcctgaccctgtcctgcgtggcctctggcttcacattttccaattacggcatgcactggatccggcaggccccaaagaagggcctggagtggatcgccatgatctactatgacagctccaagatgaactatgccgataccgtgaagggccggttcacaatcagccgcgacaactccaagaataccctgtacctggagatgaacagcctgcgctctgaggacaccgccatgtactattgtgccgtgcccacaagccactatgtggtggacgtgtggggacagggcgtgtccgtgaccgtgtctagcggaggaggaggatccggaggaggaggatctggaggaggaggatcctctgagacacaggccaacagcaccacagacgccctgaatgtgctgctgatcatcgtggacgatctgcggccctccctgggatgctacggcgacaagctggtgcgctctcctaacatcgatcagctggccagccactccctgctgttccagaatgcctttgcccagcaggccgtgtgcgcaccaagccgggtgtccttcctgaccggcaggaggcccgacaccacacggctgtacgacttcaactcttattggcgcgtgcacgccggcaatttcagcaccatccctcagtactttaaggagaacggctatgtgacaatgagcgtgggcaaggtgttccacccaggcatcagctccaatcacacagacgattccccttactcttggagctttcccccttatcacccatctagcgagaagtacgagaacaccaagacatgcaggggacctgacggagagctgcacgcaaatctgctgtgcccagtggacgtgctggatgtgccagagggcaccctgcccgataagcagagcacagagcaggccatccagctgctggagaagatgaagacctccgcctctcccttctttctggccgtgggctaccacaagccacacatccccttcagatatccaaaggagtttcagaagctgtaccccctggagaacatcacactggcaccagaccctgaggtgccagatggcctgccacccgtggcctataacccttggatggacatccggcagcgcgaggatgtgcaggccctgaatatctctgtgccttacggcccaatccccgtggacttccagcggaagatccgccagagctactttgccagcgtgtcctatctggatacccaagtgggccgcctgctgtccgccctggacgatctgcagctggccaactccaccatcatcgccttcacatctgaccacggatgggcactgggagagcacggagagtgggccaagtattctaatttcgatgtggccacccacgtgcctctgatcttttacgtgccaggaaggacagcctccctgcctgaggcaggagagaagctgttcccctacctggacccttttgattctgccagccagctgatggagccaggccgccagagcatggacctggtggagctggtgtccctgttccccaccctggcaggcctggcaggcctgcaggtgcctccaaggtgccctgtgcccagcttccacgtggagctgtgcagagagggcaagaacctgctgaagcacttcaggttcagggacctggaggaggatccttacctgccaggcaatcccagggagctgatcgcctacagccagtatcccagaccttccgacatcccccagtggaactctgacaagcctagcctgaaggatatcaagatcatgggctattccatcaggaccatcgattacagatatacagtgtgggtgggcttcaacccagacgagttcctggccaatttttctgatatccacgccggcgagctgtactttgtggacagcgatcccctgcaggaccacaatatgtataacgactcccaggggggcgatctgttccagctgctgatgccatgaaagcttatcgataccgtcgacctcgagcctgcaggcgcgtctggaacaatcaacctctggattacaaaatttgtgaaagattgactggtattcttaactatgttgctccttttacgctatgtggatacgctgctttaatgcctttgtatcatgctattgcttcccgtatggctttcattttctcctccttgtataaatcctggttgctgtctctttatgaggagttgtggcccgttgtcaggcaacgtggcgtggtgtgcactgtgtttgctgacgcaacccccactggttggggcattgccaccacctgtcagctcctttccgggactttcgctttccccctccctattgccacggcggaactcatcgccgcctgccttgcccgctgctggacaggggctcggctgttgggcactgacaattccgtggtgttgtcggggaagctgacgtcctttccatggctagctcgcctgtgttgccacctggattctgcgcgggacgtccttctgctacgtcccttcggccctcaatccagcggaccttccttcccgcggcctgctgccggctctgcggcctcttccgcgtcttcgccttcgccctcagacgagtcggatctccctttgggccgcctccccgcctggaattaattctgcagtcgagacctagaaaaacatggagcaatcacaagtagcaatacagcagctaccaatgctgattgtgcctggctagaagcacaagaggaggaggaggtgggttttccagtcacacctcaggtacctttaagaccaatgacttacaaggcagctgtagatcttagccactttttaaaagaaaagaggggactggaagggctaattcactcccaacgaagacaagattctagagggacagcccccccccaaagcccccagggatgtaattacgtccctcccccgctagggggcagcagcgagccgcccggggctccgctccggtccggcgctccccccgcatccccgagccggcagcgtgcggggacagcccgggcacggggaaggtggcacgggatcgctttcctctgaacgcttctcgctgctctttgagcctgcagacacctggggggatacggggaaaaagcttctgctttttgcttgtactgggtctctctggttagaccagatctgagcctgggagctctctggctaactagggaacccactgcttaagcctcaataaagcttgccttgagtgcttcaagtagtgtgtgcccgtctgttgtgtgactctggtaactagagatccctcagacccttttagtcagtgtggaaaatctctagcagtagtagttcatgtcatcttattattcagtatttataacttgcaaagaaatgaatatcagagagtgagaggccttgacattgctagcgttttaccgtcgacctctagctagagcttggcgtaatcatggtcatagctgtttcctgtgtgaaattgttatccgctcacaattccacacaacatacgagccggaagcataaagtgtaaagcctggggtgcctaatgagtgagctaactcacattaattgcgttgcgctcactgcccgctttccagtcgggaaacctgtcgtgccagctgcattaatgaatcggccaacgcgcggggagaggcggtttgcgtattgggcgctcttccgcttcctcgctcactgactcgctgcgctcggtcgttcggctgcggcgagcggtatcagctcactcaaaggcggtaatacggttatccacagaatcaggggataacgcaggaaagaacatgtgagcaaaaggccagcaaaaggccaggaaccgtaaaaaggccgcgttgctggcgtttttccataggctccgcccccctgacgagcatcacaaaaatcgacgctcaagtcagaggtggcgaaacccgacaggactataaagataccaggcgtttccccctggaagctccctcgtgcgctctcctgttccgaccctgccgcttaccggatacctgtccgcctttctcccttcgggaagcgtggcgctttctcatagctcacgctgtaggtatctcagttcggtgtaggtcgttcgctccaagctgggctgtgtgcacgaaccccccgttcagcccgaccgctgcgccttatccggtaactatcgtcttgagtccaacccggtaagacacgacttatcgccactggcagcagccactggtaacaggattagcagagcgaggtatgtaggcggtgctacagagttcttgaagtggtggcctaactacggctacactagaagaacagtatttggtatctgcgctctgctgaagccagttaccttcggaaaaagagttggtagctcttgatccggcaaacaaaccaccgctggtagcggtggtttttttgtttgcaagcagcagattacgcgcagaaaaaaaggatctcaagaagatcctttgatcttttctacggggtctgacgctcagtggaacgaaaactcacgttaagggattttggtcatgagattatcaaaaaggatcttcacctagatccttttaaattaaaaatgaagttttaaatcaatctaaagtatatatgagtaaacttggtctgacagttaccaatgcttaatcagtgaggcacctatctcagcgatctgtctatttcgttcatccatagttgcctgactccccgtcgtgtagataactacgatacgggagggcttaccatctggccccagtgctgcaatgataccgcgagacccacgctcaccggctccagatttatcagcaataaaccagccagccggaagggccgagcgcagaagtggtcctgcaactttatccgcctccatccagtctattaattgttgccgggaagctagagtaagtagttcgccagttaatagtttgcgcaacgttgttgccattgctacaggcatcgtggtgtcacgctcgtcgtttggtatggcttcattcagctccggttcccaacgatcaaggcgagttacatgatcccccatgttgtgcaaaaaagcggttagctccttcggtcctccgatcgttgtcagaagtaagttggccgcagtgttatcactcatggttatggcagcactgcataattctcttactgtcatgccatccgtaagatgcttttctgtgactggtgagtactcaaccaagtcattctgagaatagtgtatgcggcgaccgagttgctcttgcccggcgtcaatacgggataataccgcgccacatagcagaactttaaaagtgctcatcattggaaaacgttcttcggggcgaaaactctcaaggatcttaccgctgttgagatccagttcgatgtaacccactcgtgcacccaactgatcttcagcatcttttactttcaccagcgtttctgggtgagcaaaaacaggaaggcaaaatgccgcaaaaaagggaataagggcgacacggaaatgttgaatactcatactcttcctttttcaatattattgaagcatttatcagggttattgtctcatgagcggatacatatttgaatgtatttagaaaaataaacaaataggggttccgcgcacatttccccgaaaagtgccacctgacgtcgacggatcgggagatcaacttgtttattgcagcttataatggttacaaataaagcaatagcatcacaaatttcacaaataaagcatttttttcactgcattctagttgtggtttgtccaaactcatcaatgtatcttatcatgtctggatcaactggataactcaagctaaccaaaatcatcccaaacttcccaccccataccctattaccactgccaattacctgtggtttcatttactctaaacctgtgattcctctgaattattttcattttaaagaaattgtatttgttaaatatgtactacaaacttagtagt

SEQ ID NO: 14 - protein, 1050 aa, synthetic construct
MGWSLILLFLVAVATRVGSEVQLVQSGAEVKKPGESLKISCKGSGYSFMNYWLGWVRQMPGKGLEWMGDIYPGGDYPTYSEKFKVQVTISADKSISTAYLQLSSLKASDTAMYYCARSGNYDEVAYWGQGTLVTVSSASTKGPSVFPLAPSSKSTSGGTAALGCLVKDYFPEPVTVSWNSGALTSGVHTFPAVLQSSGLYSLSSVVTVPSSSLGTQTYICNVNHKPSNTKVDKKVEPKSCDKTHTGGGGSGGGGSGGGGSSETQANSTTDALNVLLIIVDDLRPSLGCYGDKLVRSPNIDQLASHSLLFQNAFAQQAVCAPSRVSFLTGRRPDTTRLYDFNSYWRVHAGNFSTIPQYFKENGYVTMSVGKVFHPGISSNHTDDSPYSWSFPPYHPSSEKYENTKTCRGPDGELHANLLCPVDVLDVPEGTLPDKQSTEQAIQLLEKMKTSASPFFLAVGYHKPHIPFRYPKEFQKLYPLENITLAPDPEVPDGLPPVAYNPWMDIRQREDVQALNISVPYGPIPVDFQRKIRQSYFASVSYLDTQVGRLLSALDDLQLANSTIIAFTSDHGWALGEHGEWAKYSNFDVATHVPLIFYVPGRTASLPEAGEKLFPYLDPFDSASQLMEPGRQSMDLVELVSLFPTLAGLAGLQVPPRCPVPSFHVELCREGKNLLKHFRFRDLEEDPYLPGNPRELIAYSQYPRPSDIPQWNSDKPSLKDIKIMGYSIRTIDYRYTVWVGFNPDEFLANFSDIHAGELYFVDSDPLQDHNMYNDSQGGDLFQLLMPCTGSGATNFSLLKQAGDVEENPGPVYTMGWSWILLFLLSVTAGVHSDIVMTQTPLSLSVTPGQPASISCRSSQSLVHSNGNTYLHWYLQKPGQSPQLLIYKVSNRFSGVPDRFSGSGSGTDFTLKISRVEAEDVGVYYCSQSTHVPWTFGQGTKVEIKRTVAAPSVFIFPPSDEQLKSGTASVVCLLNNFYPREAKVQWKVDNALQSGNSQESVTEQDSKDSTYSLSSTLTLSKADYEKHKVYACEVTHQGLSSPVTKSFNRGEC

SEQ ID NO: 15 - DNA, 3153 bp, synthetic construct
  source 1..3153: mol_type = other DNA
atgggttggagcctcatcttgctcttccttgtcgctgttgctacgcgagtcggcagcgaggtgcaactagtgcagtctggagcagaggtgaaaaagcccggggagtctctgaagatttcctgtaagggttctggatacagctttatgaactactggctgggatgggtgcgccagatgcccgggaaaggcctggagtggatgggggacatctaccccggcggagactaccctacatacagcgagaagttcaaggtccaggtcaccatctcagccgacaagtccatcagcaccgcctacctgcagttgagcagcctgaaggcctcggacaccgccatgtattactgtgcgagatcaggcaattacgacgaagtggcctactggggccaaggaaccctggtcaccgtctcctcagctagcaccaagggcccatcggtcttccccctggcaccctcctccaagagcacctctgggggcacagcggccctgggctgcctggtcaaggactacttccccgaaccggtgacggtgtcgtggaactcaggcgccctgaccagcggcgtgcacaccttcccggctgtcctacagtcctcaggactctactccctcagcagcgtggtgaccgtgccctccagcagcttgggcacccagacctacatctgcaacgtgaatcacaagcccagcaacaccaaggtggacaagaaagttgagccgaagagctgtgataagacgcatacgggtggcggagggtctggaggtggcggatcaggcggaggtggatcttccgaaacgcaggccaactcgaccacagatgctctgaacgttcttctcatcatcgtggatgacctgcgcccctccctgggctgttatggggataagctggtgaggtccccaaatattgaccaactggcatcccacagcctcctcttccagaatgcctttgcgcagcaagcagtgtgcgccccgagccgcgtttctttcctcactggcaggagacctgacaccacccgcctgtacgacttcaactcctactggagggtgcacgctggaaacttctccaccatcccccagtacttcaaggagaatggctatgtgaccatgtcggtgggaaaagtctttcaccctgggatatcttctaaccataccgatgattctccgtatagctggtcttttccaccttatcatccttcctctgagaagtatgaaaacactaagacatgtcgagggccagatggagaactccatgccaacctgctttgccctgtggatgtgctggatgttcccgagggcaccttgcctgacaaacagagcactgagcaagccatacagttgttggaaaagatgaaaacgtcagccagtcctttcttcctggccgttgggtatcataagccacacatccccttcagataccccaaggaatttcagaagttgtatcccttggagaacatcaccctggcccccgatcccgaggtccctgatggcctaccccctgtggcctacaacccctggatggacatcaggcaacgggaagacgtccaagccttaaacatcagtgtgccgtatggtccaattcctgtggactttcagcggaaaatccgccagagctactttgcctctgtgtcatatttggatacacaggtcggccgcctcttgagtgctttggacgatcttcagctggccaacagcaccatcattgcatttacctcggatcatgggtgggctctaggtgaacatggagaatgggccaaatacagcaattttgatgttgctacccatgttcccctgatattctatgttcctggaaggacggcttcacttccggaggcaggcgagaagcttttcccttacctcgacccttttgattccgcctcacagttgatggagccaggcaggcaatccatggaccttgtggaacttgtgtctctttttcccacgctggctggacttgcaggactgcaggttccacctcgctgccccgttccttcatttcacgttgagctgtgcagagaaggcaagaaccttctgaagcattttcgattccgtgacttggaagaagatccgtacctccctggtaatccccgtgaactgattgcctatagccagtatccccggccttcagacatccctcagtggaattctgacaagccgagtttaaaagatataaagatcatgggctattccatacgcaccatagactataggtatactgtgtgggttggcttcaatcctgatgaatttctagctaacttttctgacatccatgcaggggaactgtattttgtggattctgacccattgcaggatcacaatatgtataatgattcccaaggtggagaccttttccagttgttgatgccttgtacaggaagcggagccacgaacttctctctgttaaagcaagcaggagacgtggaagaaaaccccggtcctgtgtacaccatgggctggagctggattctgctgttcctcctgagcgtgacagcaggagtgcacagcgacatcgtgatgacccagactcccctgagcctgagcgtgacacctggccagcctgccagcatcagctgcagaagctctcagagcctggtgcacagcaacggcaacacctacctgcactggtatctgcagaagcccggccagagccctcagctgctgatctacaaggtgtccaacagattcagcggcgtgcccgacagattctccggcagcggctctggcaccgacttcaccctgaagatttccagagtggaagccgaggacgtgggcgtgtactactgcagccagagcacccacgtgccctggacattcggccagggcaccaaggtggaaatcaagagaaccgtggccgctcccagcgtgttcatcttcccacctagcgacgagcagctgaagtccggcacagcctctgtcgtgtgcctgctgaacaacttctacccccgcgaggccaaggtgcagtggaaggtggacaacgccctgcagagcggcaacagccaggaaagcgtgaccgagcaggactccaaggacagcacctacagcctgagcagcaccctgaccctgagcaaggccgactacgagaagcacaaggtgtacgcctgcgaagtgacccaccagggcctgtctagccccgtgaccaagagcttcaacagaggcgagtgctaa

SEQ ID NO: 16 - DNA, 9611 bp, synthetic construct
  source 1..9611: mol_type = other DNA
gaattctaatagtaatcaattacggggtcattagttcatagcccatatatggagttccgcgttacataacttacggtaaatggcccgcctggctgaccgcccaacgacccccgcccattgacgtcaataatgacgtatgttcccatagtaacgccaatagggactttccattgacgtcaatgggtggagtatttacggtaaactgcccacttggcagtacatcaagtgtatcatatgccaagtacgccccctattgacgtcaatgacggtaaatggcccgcctggcattatgcccagtacatgaccttatgggactttcctacttggcagtacatctacgtattagtcatcgctattaccatggtgatgcggttttggcagtacatcaatgggcgtggatagcggtttgactcacggggatttccaagtctccaccccattgacgtcaatgggagtttgttttggcaccaaaatcaacgggactttccaaaatgtcgtaacaactccgccccattgacgcaaatgggcggtaggcgtgtacggtgggaggtctatataagcagagctggtttagtgaaccgggtctctctggttagaccagatctgagcctgggagctctctggctaactagggaacccactgcttaagcctcaataaagcttgccttgagtgcttcaagtagtgtgtgcccgtctgttgtgtgactctggtaactagagatccctcagacccttttagtcagtgtggaaaatctctagcagtggcgcccgaacagggacttgaaagcgaaagggaaaccagaggagctctctcgacgcaggactcggcttgctgaagcgcgcacggcaagaggcgaggggcggcgactggtgagtacgccaaaaattttgactagcggaggctagaaggagagagatgggtgcgagagcgtcagtattaagcgggggagaattagatcgcgatgggaaaaaattcggttaaggccagggggaaagaaaaaatataaattaaaacatatagtatgggcaagcagggagctagaacgattcgcagttaatcctggcctgttagaaacatcagaaggctgtagacaaatacgccgctgatcttcagacctggaggaggagatatgagggacaattggagaagtgaattatataaatataaagtagtaaaaattgaaccattaggagtagcacccaccaaggcaaagagaagagtggtgcagagagaaaaaagagcagtgggaataggagctttgttccttgggttcttgggagcagcaggaagcactatgggcgcagcgtcaatgacgctgacggtacaggccagacaattattgtctggtatagtgcagcagcagaacaatttgctgagggctattgaggcgcaacagcatctgttgcaactcacagtctggggcatcaagcagctccaggcaagaatcctggctgtggaaagatacctaaaggatcaacagctcctggggatttggggttgctctggaaaactcatttgcaccactgctgtgccttggaatgctagttggagtaataaatctctggaacagatttggaatcacacgacctggatggagtgggacagagaaattaacaattacacaagcttaatacactccttaattgaagaatcgcaaaaccagcaagaaaagaatgaacaagaattattggaattagataaatgggcaagtttgtggaattggtttaacataacaaattggctgtggtatataaaattattcataatgatagtaggaggcttggtaggtttaagaatagtttttgctgtactttctatagtgaatagagttaggcagggatattcaccattatcgtttcagacccacctcccaaccccgaggggacccgacaggcccgaaggaatagaagaagaaggtggagagagagacagagacagatccattcgattagtgaacggatctcgacggtatcgcctttaaaagaaaaggggggattggggggtacagtgcaggggaaagaatagtagacataatagcaacagacatacaaactaaagaattacaaaaacaaattacaaaaattcaaaattttcgggtttattacagggacagcagagatccagtttatcgatttaaatacgcgtgggaatgaaagaccccacctgtaggtttggcaagctaggatcaaggtcaggaacagagaaacaggagaatatgggccaaacaggatatctgtggtaagcagttcctgccccgctcagggccaagaacagttggaacaggagaatatgggccaaacaggatatctgtggtaagcagttcctgccccgctcagggccaagaacagatggtccccagatgcggtcccgccctcagcagtttctagagaaccatcagatgtttccagggtgccccaaggacctgaaatgaccctgtgccttatttgaactaaccaatcagttcgcttctcgcttctgttcgcgcgcttctgctccccgagctctatataagcagagctggtttagtgaaccgtcagatcggatccgcgtgccaccatgggttggagcctcatcttgctcttccttgtcgctgttgctacgcgagtcggcagcgaggtgcaactagtgcagtctggagcagaggtgaaaaagcccggggagtctctgaagatttcctgtaagggttctggatacagctttatgaactactggctgggatgggtgcgccagatgcccgggaaaggcctggagtggatgggggacatctaccccggcggagactaccctacatacagcgagaagttcaaggtccaggtcaccatctcagccgacaagtccatcagcaccgcctacctgcagttgagcagcctgaaggcctcggacaccgccatgtattactgtgcgagatcaggcaattacgacgaagtggcctactggggccaaggaaccctggtcaccgtctcctcagctagcaccaagggcccatcggtcttccccctggcaccctcctccaagagcacctctgggggcacagcggccctgggctgcctggtcaaggactacttccccgaaccggtgacggtgtcgtggaactcaggcgccctgaccagcggcgtgcacaccttcccggctgtcctacagtcctcaggactctactccctcagcagcgtggtgaccgtgccctccagcagcttgggcacccagacctacatctgcaacgtgaatcacaagcccagcaacaccaaggtggacaagaaagttgagccgaagagctgtgataagacgcatacgggtggcggagggtctggaggtggcggatcaggcggaggtggatcttccgaaacgcaggccaactcgaccacagatgctctgaacgttcttctcatcatcgtggatgacctgcgcccctccctgggctgttatggggataagctggtgaggtccccaaatattgaccaactggcatcccacagcctcctcttccagaatgcctttgcgcagcaagcagtgtgcgccccgagccgcgtttctttcctcactggcaggagacctgacaccacccgcctgtacgacttcaactcctactggagggtgcacgctggaaacttctccaccatcccccagtacttcaaggagaatggctatgtgaccatgtcggtgggaaaagtctttcaccctgggatatcttctaaccataccgatgattctccgtatagctggtcttttccaccttatcatccttcctctgagaagtatgaaaacactaagacatgtcgagggccagatggagaactccatgccaacctgctttgccctgtggatgtgctggatgttcccgagggcaccttgcctgacaaacagagcactgagcaagccatacagttgttggaaaagatgaaaacgtcagccagtcctttcttcctggccgttgggtatcataagccacacatccccttcagataccccaaggaatttcagaagttgtatcccttggagaacatcaccctggcccccgatcccgaggtccctgatggcctaccccctgtggcctacaacccctggatggacatcaggcaacgggaagacgtccaagccttaaacatcagtgtgccgtatggtccaattcctgtggactttcagcggaaaatccgccagagctactttgcctctgtgtcatatttggatacacaggtcggccgcctcttgagtgctttggacgatcttcagctggccaacagcaccatcattgcatttacctcggatcatgggtgggctctaggtgaacatggagaatgggccaaatacagcaattttgatgttgctacccatgttcccctgatattctatgttcctggaaggacggcttcacttccggaggcaggcgagaagcttttcccttacctcgacccttttgattccgcctcacagttgatggagccaggcaggcaatccatggaccttgtggaacttgtgtctctttttcccacgctggctggacttgcaggactgcaggttccacctcgctgccccgttccttcatttcacgttgagctgtgcagagaaggcaagaaccttctgaagcattttcgattccgtgacttggaagaagatccgtacctccctggtaatccccgtgaactgattgcctatagccagtatccccggccttcagacatccctcagtggaattctgacaagccgagtttaaaagatataaagatcatgggctattccatacgcaccatagactataggtatactgtgtgggttggcttcaatcctgatgaatttctagctaacttttctgacatccatgcaggggaactgtattttgtggattctgacccattgcaggatcacaatatgtataatgattcccaaggtggagaccttttccagttgttgatgccttgtacaggaagcggagccacgaacttctctctgttaaagcaagcaggagacgtggaagaaaaccccggtcctgtgtacaccatgggctggagctggattctgctgttcctcctgagcgtgacagcaggagtgcacagcgacatcgtgatgacccagactcccctgagcctgagcgtgacacctggccagcctgccagcatcagctgcagaagctctcagagcctggtgcacagcaacggcaacacctacctgcactggtatctgcagaagcccggccagagccctcagctgctgatctacaaggtgtccaacagattcagcggcgtgcccgacagattctccggcagcggctctggcaccgacttcaccctgaagatttccagagtggaagccgaggacgtgggcgtgtactactgcagccagagcacccacgtgccctggacattcggccagggcaccaaggtggaaatcaagagaaccgtggccgctcccagcgtgttcatcttcccacctagcgacgagcagctgaagtccggcacagcctctgtcgtgtgcctgctgaacaacttctacccccgcgaggccaaggtgcagtggaaggtggacaacgccctgcagagcggcaacagccaggaaagcgtgaccgagcaggactccaaggacagcacctacagcctgagcagcaccctgaccctgagcaaggccgactacgagaagcacaaggtgtacgcctgcgaagtgacccaccagggcctgtctagccccgtgaccaagagcttcaacagaggcgagtgctaactcgagcctgcaggcgcgtctggaacaatcaacctctggattacaaaatttgtgaaagattgactggtattcttaactatgttgctccttttacgctatgtggatacgctgctttaatgcctttgtatcatgctattgcttcccgtatggctttcattttctcctccttgtataaatcctggttgctgtctctttatgaggagttgtggcccgttgtcaggcaacgtggcgtggtgtgcactgtgtttgctgacgcaacccccactggttggggcattgccaccacctgtcagctcctttccgggactttcgctttccccctccctattgccacggcggaactcatcgccgcctgccttgcccgctgctggacaggggctcggctgttgggcactgacaattccgtggtgttgtcggggaagctgacgtcctttccatggctagctcgcctgtgttgccacctggattctgcgcgggacgtccttctgctacgtcccttcggccctcaatccagcggaccttccttcccgcggcctgctgccggctctgcggcctcttccgcgtcttcgccttcgccctcagacgagtcggatctccctttgggccgcctccccgcctggaattaattctgcagtcgagacctagaaaaacatggagcaatcacaagtagcaatacagcagctaccaatgctgattgtgcctggctagaagcacaagaggaggaggaggtgggttttccagtcacacctcaggtacctttaagaccaatgacttacaaggcagctgtagatcttagccactttttaaaagaaaagaggggactggaagggctaattcactcccaacgaagacaagattctagagggacagcccccccccaaagcccccagggatgtaattacgtccctcccccgctagggggcagcagcgagccgcccggggctccgctccggtccggcgctccccccgcatccccgagccggcagcgtgcggggacagcccgggcacggggaaggtggcacgggatcgctttcctctgaacgcttctcgctgctctttgagcctgcagacacctggggggatacggggaaaaagcttctgctttttgcttgtactgggtctctctggttagaccagatctgagcctgggagctctctggctaactagggaacccactgcttaagcctcaataaagcttgccttgagtgcttcaagtagtgtgtgcccgtctgttgtgtgactctggtaactagagatccctcagacccttttagtcagtgtggaaaatctctagcagtagtagttcatgtcatcttattattcagtatttataacttgcaaagaaatgaatatcagagagtgagaggccttgacattgctagcgttttaccgtcgacctctagctagagcttggcgtaatcatggtcatagctgtttcctgtgtgaaattgttatccgctcacaattccacacaacatacgagccggaagcataaagtgtaaagcctggggtgcctaatgagtgagctaactcacattaattgcgttgcgctcactgcccgctttccagtcgggaaacctgtcgtgccagctgcattaatgaatcggccaacgcgcggggagaggcggtttgcgtattgggcgctcttccgcttcctcgctcactgactcgctgcgctcggtcgttcggctgcggcgagcggtatcagctcactcaaaggcggtaatacggttatccacagaatcaggggataacgcaggaaagaacatgtgagcaaaaggccagcaaaaggccaggaaccgtaaaaaggccgcgttgctggcgtttttccataggctccgcccccctgacgagcatcacaaaaatcgacgctcaagtcagaggtggcgaaacccgacaggactataaagataccaggcgtttccccctggaagctccctcgtgcgctctcctgttccgaccctgccgcttaccggatacctgtccgcctttctcccttcgggaagcgtggcgctttctcatagctcacgctgtaggtatctcagttcggtgtaggtcgttcgctccaagctgggctgtgtgcacgaaccccccgttcagcccgaccgctgcgccttatccggtaactatcgtcttgagtccaacccggtaagacacgacttatcgccactggcagcagccactggtaacaggattagcagagcgaggtatgtaggcggtgctacagagttcttgaagtggtggcctaactacggctacactagaagaacagtatttggtatctgcgctctgctgaagccagttaccttcggaaaaagagttggtagctcttgatccggcaaacaaaccaccgctggtagcggtggtttttttgtttgcaagcagcagattacgcgcagaaaaaaaggatctcaagaagatcctttgatcttttctacggggtctgacgctcagtggaacgaaaactcacgttaagggattttggtcatgagattatcaaaaaggatcttcacctagatccttttaaattaaaaatgaagttttaaatcaatctaaagtatatatgagtaaacttggtctgacagttaccaatgcttaatcagtgaggcacctatctcagcgatctgtctatttcgttcatccatagttgcctgactccccgtcgtgtagataactacgatacgggagggcttaccatctggccccagtgctgcaatgataccgcgagacccacgctcaccggctccagatttatcagcaataaaccagccagccggaagggccgagcgcagaagtggtcctgcaactttatccgcctccatccagtctattaattgttgccgggaagctagagtaagtagttcgccagttaatagtttgcgcaacgttgttgccattgctacaggcatcgtggtgtcacgctcgtcgtttggtatggcttcattcagctccggttcccaacgatcaaggcgagttacatgatcccccatgttgtgcaaaaaagcggttagctccttcggtcctccgatcgttgtcagaagtaagttggccgcagtgttatcactcatggttatggcagcactgcataattctcttactgtcatgccatccgtaagatgcttttctgtgactggtgagtactcaaccaagtcattctgagaatagtgtatgcggcgaccgagttgctcttgcccggcgtcaatacgggataataccgcgccacatagcagaactttaaaagtgctcatcattggaaaacgttcttcggggcgaaaactctcaaggatcttaccgctgttgagatccagttcgatgtaacccactcgtgcacccaactgatcttcagcatcttttactttcaccagcgtttctgggtgagcaaaaacaggaaggcaaaatgccgcaaaaaagggaataagggcgacacggaaatgttgaatactcatactcttcctttttcaatattattgaagcatttatcagggttattgtctcatgagcggatacatatttgaatgtatttagaaaaataaacaaataggggttccgcgcacatttccccgaaaagtgccacctgacgtcgacggatcgggagatcaacttgtttattgcagcttataatggttacaaataaagcaatagcatcacaaatttcacaaataaagcatttttttcactgcattctagttgtggtttgtccaaactcatcaatgtatcttatcatgtctggatcaactggataactcaagctaaccaaaatcatcccaaacttcccaccccataccctattaccactgccaattacctgtggtttcatttactctaaacctgtgattcctctgaattattttcattttaaagaaattgtatttgttaaatatgtactacaaacttagtagt

SEQ ID NO: 17 - protein, 952 aa, synthetic construct
MGVRHPPCSHRLLAVCALVSLATAALLGHILLHDFLLVPRELSGSSPVLEETHPAHQQGASRPGPRDAQAHPGRPRAVPTQCDVPPNSRFDCAPDKAITQEQCEARGCCYIPAKQGLQGAQMGQPWCFFPPSYPSYKLENLSSSEMGYTATLTRTTPTFFPKDILTLRLDVMMETENRLHFTIKDPANRRYEVPLETPRVHSRAPSPLYSVEFSEEPFGVIVHRQLDGRVLLNTTVAPLFFADQFLQLSTSLPSQYITGLAEHLSPLMLSTSWTRITLWNRDLAPTPGANLYGSHPFYLALEDGGSAHGVFLLNSNAMDVVLQPSPALSWRSTGGILDVYIFLGPEPKSVVQQYLDVVGYPFMPPYWGLGFHLCRWGYSSTAITRQVVENMTRAHFPLDVQWNDLDYMDSRRDFTFNKDGFRDFPAMVQELHQGGRRYMMIVDPAISSSGPAGSYRPYDEGLRRGVFITNETGQPLIGKVWPGSTAFPDFTNPTALAWWEDMVAEFHDQVPFDGMWIDMNEPSNFIRGSEDGCPNNELENPPYVPGVVGGTLQAATICASSHQFLSTHYNLHNLYGLTEAIASHRALVKARGTRPFVISRSTFAGHGRYAGHWTGDVWSSWEQLASSVPEILQFNLLGVPLVGADVCGFLGNTSEELCVRWTQLGAFYPFMRNHNSLLSLPQEPYSFSEPAQQAMRKALTLRYALLPHLYTLFHQAHVAGETVARPLFLEFPKDSSTWTVDHQLLWGEALLITPVLQAGKAEVTGYFPLGTWYDLQTVPIEALGSLPPPPAAPREPAIHSEGQWVTLPAPLDTINVHLRAGYIIPLQGPGLTTTESRQQPMALAVALTKGGEARGELFWDDGESLEVLERGAYTQVIFLARNNTIVNELVRVTSEGAGLQLQKVTVLGVATAPQQVLSNGVPVSNFTYSPDTKVLDICVSLLMGEQFLVSWC

SEQ ID NO: 18 - DNA, 2859 bp, synthetic construct
  source 1..2859: mol_type = other DNA
atgggagtgaggcacccgccctgctcccaccggctcctggccgtctgcgccctcgtgtccttggcaaccgctgcactcctggggcacatcctactccatgatttcctgctggttccccgagagctgagtggctcctccccagtcctggaggagactcacccagctcaccagcagggagccagcagaccagggccccgggatgcccaggcacaccccggccgtcccagagcagtgcccacacagtgcgacgtcccccccaacagccgcttcgattgcgcccctgacaaggccatcacccaggaacagtgcgaggcccgcggctgttgctacatccctgcaaagcaggggctgcagggagcccagatggggcagccctggtgcttcttcccacccagctaccccagctacaagctggagaacctgagctcctctgaaatgggctacacggccaccctgacccgtaccacccccaccttcttccccaaggacatcctgaccctgcggctggacgtgatgatggagactgagaaccgcctccacttcacgatcaaagatccagctaacaggcgctacgaggtgcccttggagaccccgcgtgtccacagccgggcaccgtccccactctacagcgtggagttctccgaggagcccttcggggtgatcgtgcaccggcagctggacggccgcgtgctgctgaacacgacggtggcgcccctgttctttgcggaccagttccttcagctgtccacctcgctgccctcgcagtatatcacaggcctcgccgagcacctcagtcccctgatgctcagcaccagctggaccaggatcaccctgtggaaccgggaccttgcgcccacgcccggtgcgaacctctacgggtctcaccctttctacctggcgctggaggacggcgggtcggcacacggggtgttcctgctaaacagcaatgccatggatgtggtcctgcagccgagccctgcccttagctggaggtcgacaggtgggatcctggatgtctacatcttcctgggcccagagcccaagagcgtggtgcagcagtacctggacgttgtgggatacccgttcatgccgccatactggggcctgggcttccacctgtgccgctggggctactcctccaccgctatcacccgccaggtggtggagaacatgaccagggcccacttccccctggacgtccagtggaacgacctggactacatggactcccggagggacttcacgttcaacaaggatggcttccgggacttcccggccatggtgcaggagctgcaccagggcggccggcgctacatgatgatcgtggatcctgccatcagcagctcgggccctgccgggagctacaggccctacgacgagggtctgcggaggggggttttcatcaccaacgagaccggccagccgctgattgggaaggtatggcccgggtccactgccttccccgacttcaccaaccccacagccctggcctggtgggaggacatggtggctgagttccatgaccaggtgcccttcgacggcatgtggattgacatgaacgagccttccaacttcatcaggggctctgaggacggctgccccaacaatgagctggagaacccaccctacgtgcctggggtggttggggggaccctccaggcggccaccatctgtgcctccagccaccagtttctctccacacactacaacctgcacaacctctacggcctgaccgaagccatcgcctcccacagggcgctggtgaaggctcgggggacacgcccatttgtgatctcccgctcgacctttgctggccacggccgatacgccggccactggacgggggacgtgtggagctcctgggagcagctcgcctcctccgtgccagaaatcctgcagtttaacctgctgggggtgcctctggtcggggccgacgtctgcggcttcctgggcaacacctcagaggagctgtgtgtgcgctggacccagctgggggccttctaccccttcatgcggaaccacaacagcctgctcagtctgccccaggagccgtacagcttcagcgagccggcccagcaggccatgaggaaggccctcaccctgcgctacgcactcctcccccacctctacacactgttccaccaggcccacgtcgcgggggagaccgtggcccggcccctcttcctggagttccccaaggactctagcacctggactgtggaccaccagctcctgtggggggaggccctgctcatcaccccagtgctccaggccgggaaggccgaagtgactggctacttccccttgggcacatggtacgacctgcagacggtgccaatagaggcccttggcagcctcccacccccacctgcagctccccgtgagccagccatccacagcgaggggcagtgggtgacgctgccggcccccctggacaccatcaacgtccacctccgggctgggtacatcatccccctgcagggccctggcctcacaaccacagagtcccgccagcagcccatggccctggctgtggccctgaccaagggtggggaggcccgaggggagctgttctgggacgatggagagagcctggaagtgctggagcgaggggcctacacacaggtcatcttcctggccaggaataacacgatcgtgaatgagctggtacgtgtgaccagtgagggagctggcctgcagctgcagaaggtgactgtcctgggcgtggccacggcgccccagcaggtcctctccaacggtgtccctgtctccaacttcacctacagccccgacaccaaggtcctggacatctgtgtctcgctgttgatgggagagcagtttctcgtcagctggtgttag

SEQ ID NO: 19 - DNA, 9324 bp, synthetic construct
  source 1..9324: mol_type = other DNA
gaattctaatagtaatcaattacggggtcattagttcatagcccatatatggagttccgcgttacataacttacggtaaatggcccgcctggctgaccgcccaacgacccccgcccattgacgtcaataatgacgtatgttcccatagtaacgccaatagggactttccattgacgtcaatgggtggagtatttacggtaaactgcccacttggcagtacatcaagtgtatcatatgccaagtacgccccctattgacgtcaatgacggtaaatggcccgcctggcattatgcccagtacatgaccttatgggactttcctacttggcagtacatctacgtattagtcatcgctattaccatggtgatgcggttttggcagtacatcaatgggcgtggatagcggtttgactcacggggatttccaagtctccaccccattgacgtcaatgggagtttgttttggcaccaaaatcaacgggactttccaaaatgtcgtaacaactccgccccattgacgcaaatgggcggtaggcgtgtacggtgggaggtctatataagcagagctggtttagtgaaccgggtctctctggttagaccagatctgagcctgggagctctctggctaactagggaacccactgcttaagcctcaataaagcttgccttgagtgcttcaagtagtgtgtgcccgtctgttgtgtgactctggtaactagagatccctcagacccttttagtcagtgtggaaaatctctagcagtggcgcccgaacagggacttgaaagcgaaagggaaaccagaggagctctctcgacgcaggactcggcttgctgaagcgcgcacggcaagaggcgaggggcggcgactggtgagtacgccaaaaattttgactagcggaggctagaaggagagagatgggtgcgagagcgtcagtattaagcgggggagaattagatcgcgatgggaaaaaattcggttaaggccagggggaaagaaaaaatataaattaaaacatatagtatgggcaagcagggagctagaacgattcgcagttaatcctggcctgttagaaacatcagaaggctgtagacaaatacgccgctgatcttcagacctggaggaggagatatgagggacaattggagaagtgaattatataaatataaagtagtaaaaattgaaccattaggagtagcacccaccaaggcaaagagaagagtggtgcagagagaaaaaagagcagtgggaataggagctttgttccttgggttcttgggagcagcaggaagcactatgggcgcagcgtcaatgacgctgacggtacaggccagacaattattgtctggtatagtgcagcagcagaacaatttgctgagggctattgaggcgcaacagcatctgttgcaactcacagtctggggcatcaagcagctccaggcaagaatcctggctgtggaaagatacctaaaggatcaacagctcctggggatttggggttgctctggaaaactcatttgcaccactgctgtgccttggaatgctagttggagtaataaatctctggaacagatttggaatcacacgacctggatggagtgggacagagaaattaacaattacacaagcttaatacactccttaattgaagaatcgcaaaaccagcaagaaaagaatgaacaagaattattggaattagataaatgggcaagtttgtggaattggtttaacataacaaattggctgtggtatataaaattattcataatgatagtaggaggcttggtaggtttaagaatagtttttgctgtactttctatagtgaatagagttaggcagggatattcaccattatcgtttcagacccacctcccaaccccgaggggacccgacaggcccgaaggaatagaagaagaaggtggagagagagacagagacagatccattcgattagtgaacggatctcgacggtatcgcctttaaaagaaaaggggggattggggggtacagtgcaggggaaagaatagtagacataatagcaacagacatacaaactaaagaattacaaaaacaaattacaaaaattcaaaattttcgggtttattacagggacagcagagatccagtttatcgatttaaatacgcgtgggaatgaaagaccccacctgtaggtttggcaagctaggatcaaggtcaggaacagagaaacaggagaatatgggccaaacaggatatctgtggtaagcagttcctgccccgctcagggccaagaacagttggaacaggagaatatgggccaaacaggatatctgtggtaagcagttcctgccccgctcagggccaagaacagatggtccccagatgcggtcccgccctcagcagtttctagagaaccatcagatgtttccagggtgccccaaggacctgaaatgaccctgtgccttatttgaactaaccaatcagttcgcttctcgcttctgttcgcgcgcttctgctccccgagctctatataagcagagctggtttagtgaaccgtcagatcggatccgcggccgcgccgccaccatgggagtgaggcacccgccctgctcccaccggctcctggccgtctgcgccctcgtgtccttggcaaccgctgcactcctggggcacatcctactccatgatttcctgctggttccccgagagctgagtggctcctccccagtcctggaggagactcacccagctcaccagcagggagccagcagaccagggccccgggatgcccaggcacaccccggccgtcccagagcagtgcccacacagtgcgacgtcccccccaacagccgcttcgattgcgcccctgacaaggccatcacccaggaacagtgcgaggcccgcggctgttgctacatccctgcaaagcaggggctgcagggagcccagatggggcagccctggtgcttcttcccacccagctaccccagctacaagctggagaacctgagctcctctgaaatgggctacacggccaccctgacccgtaccacccccaccttcttccccaaggacatcctgaccctgcggctggacgtgatgatggagactgagaaccgcctccacttcacgatcaaagatccagctaacaggcgctacgaggtgcccttggagaccccgcgtgtccacagccgggcaccgtccccactctacagcgtggagttctccgaggagcccttcggggtgatcgtgcaccggcagctggacggccgcgtgctgctgaacacgacggtggcgcccctgttctttgcggaccagttccttcagctgtccacctcgctgccctcgcagtatatcacaggcctcgccgagcacctcagtcccctgatgctcagcaccagctggaccaggatcaccctgtggaaccgggaccttgcgcccacgcccggtgcgaacctctacgggtctcaccctttctacctggcgctggaggacggcgggtcggcacacggggtgttcctgctaaacagcaatgccatggatgtggtcctgcagccgagccctgcccttagctggaggtcgacaggtgggatcctggatgtctacatcttcctgggcccagagcccaagagcgtggtgcagcagtacctggacgttgtgggatacccgttcatgccgccatactggggcctgggcttccacctgtgccgctggggctactcctccaccgctatcacccgccaggtggtggagaacatgaccagggcccacttccccctggacgtccagtggaacgacctggactacatggactcccggagggacttcacgttcaacaaggatggcttccgggacttcccggccatggtgcaggagctgcaccagggcggccggcgctacatgatgatcgtggatcctgccatcagcagctcgggccctgccgggagctacaggccctacgacgagggtctgcggaggggggttttcatcaccaacgagaccggccagccgctgattgggaaggtatggcccgggtccactgccttccccgacttcaccaaccccacagccctggcctggtgggaggacatggtggctgagttccatgaccaggtgcccttcgacggcatgtggattgacatgaacgagccttccaacttcatcaggggctctgaggacggctgccccaacaatgagctggagaacccaccctacgtgcctggggtggttggggggaccctccaggcggccaccatctgtgcctccagccaccagtttctctccacacactacaacctgcacaacctctacggcctgaccgaagccatcgcctcccacagggcgctggtgaaggctcgggggacacgcccatttgtgatctcccgctcgacctttgctggccacggccgatacgccggccactggacgggggacgtgtggagctcctgggagcagctcgcctcctccgtgccagaaatcctgcagtttaacctgctgggggtgcctctggtcggggccgacgtctgcggcttcctgggcaacacctcagaggagctgtgtgtgcgctggacccagctgggggccttctaccccttcatgcggaaccacaacagcctgctcagtctgccccaggagccgtacagcttcagcgagccggcccagcaggccatgaggaaggccctcaccctgcgctacgcactcctcccccacctctacacactgttccaccaggcccacgtcgcgggggagaccgtggcccggcccctcttcctggagttccccaaggactctagcacctggactgtggaccaccagctcctgtggggggaggccctgctcatcaccccagtgctccaggccgggaaggccgaagtgactggctacttccccttgggcacatggtacgacctgcagacggtgccaatagaggcccttggcagcctcccacccccacctgcagctccccgtgagccagccatccacagcgaggggcagtgggtgacgctgccggcccccctggacaccatcaacgtccacctccgggctgggtacatcatccccctgcagggccctggcctcacaaccacagagtcccgccagcagcccatggccctggctgtggccctgaccaagggtggggaggcccgaggggagctgttctgggacgatggagagagcctggaagtgctggagcgaggggcctacacacaggtcatcttcctggccaggaataacacgatcgtgaatgagctggtacgtgtgaccagtgagggagctggcctgcagctgcagaaggtgactgtcctgggcgtggccacggcgccccagcaggtcctctccaacggtgtccctgtctccaacttcacctacagccccgacaccaaggtcctggacatctgtgtctcgctgttgatgggagagcagtttctcgtcagctggtgttagctcgagcctgcaggcgcgtctggaacaatcaacctctggattacaaaatttgtgaaagattgactggtattcttaactatgttgctccttttacgctatgtggatacgctgctttaatgcctttgtatcatgctattgcttcccgtatggctttcattttctcctccttgtataaatcctggttgctgtctctttatgaggagttgtggcccgttgtcaggcaacgtggcgtggtgtgcactgtgtttgctgacgcaacccccactggttggggcattgccaccacctgtcagctcctttccgggactttcgctttccccctccctattgccacggcggaactcatcgccgcctgccttgcccgctgctggacaggggctcggctgttgggcactgacaattccgtggtgttgtcggggaagctgacgtcctttccatggctagctcgcctgtgttgccacctggattctgcgcgggacgtccttctgctacgtcccttcggccctcaatccagcggaccttccttcccgcggcctgctgccggctctgcggcctcttccgcgtcttcgccttcgccctcagacgagtcggatctccctttgggccgcctccccgcctggaattaattctgcagtcgagacctagaaaaacatggagcaatcacaagtagcaatacagcagctaccaatgctgattgtgcctggctagaagcacaagaggaggaggaggtgggttttccagtcacacctcaggtacctttaagaccaatgacttacaaggcagctgtagatcttagccactttttaaaagaaaagaggggactggaagggctaattcactcccaacgaagacaagattctagagggacagcccccccccaaagcccccagggatgtaattacgtccctcccccgctagggggcagcagcgagccgcccggggctccgctccggtccggcgctccccccgcatccccgagccggcagcgtgcggggacagcccgggcacggggaaggtggcacgggatcgctttcctctgaacgcttctcgctgctctttgagcctgcagacacctggggggatacggggaaaaagcttctgctttttgcttgtactgggtctctctggttagaccagatctgagcctgggagctctctggctaactagggaacccactgcttaagcctcaataaagcttgccttgagtgcttcaagtagtgtgtgcccgtctgttgtgtgactctggtaactagagatccctcagacccttttagtcagtgtggaaaatctctagcagtagtagttcatgtcatcttattattcagtatttataacttgcaaagaaatgaatatcagagagtgagaggccttgacattgctagcgttttaccgtcgacctctagctagagcttggcgtaatcatggtcatagctgtttcctgtgtgaaattgttatccgctcacaattccacacaacatacgagccggaagcataaagtgtaaagcctggggtgcctaatgagtgagctaactcacattaattgcgttgcgctcactgcccgctttccagtcgggaaacctgtcgtgccagctgcattaatgaatcggccaacgcgcggggagaggcggtttgcgtattgggcgctcttccgcttcctcgctcactgactcgctgcgctcggtcgttcggctgcggcgagcggtatcagctcactcaaaggcggtaatacggttatccacagaatcaggggataacgcaggaaagaacatgtgagcaaaaggccagcaaaaggccaggaaccgtaaaaaggccgcgttgctggcgtttttccataggctccgcccccctgacgagcatcacaaaaatcgacgctcaagtcagaggtggcgaaacccgacaggactataaagataccaggcgtttccccctggaagctccctcgtgcgctctcctgttccgaccctgccgcttaccggatacctgtccgcctttctcccttcgggaagcgtggcgctttctcatagctcacgctgtaggtatctcagttcggtgtaggtcgttcgctccaagctgggctgtgtgcacgaaccccccgttcagcccgaccgctgcgccttatccggtaactatcgtcttgagtccaacccggtaagacacgacttatcgccactggcagcagccactggtaacaggattagcagagcgaggtatgtaggcggtgctacagagttcttgaagtggtggcctaactacggctacactagaagaacagtatttggtatctgcgctctgctgaagccagttaccttcggaaaaagagttggtagctcttgatccggcaaacaaaccaccgctggtagcggtggtttttttgtttgcaagcagcagattacgcgcagaaaaaaaggatctcaagaagatcctttgatcttttctacggggtctgacgctcagtggaacgaaaactcacgttaagggattttggtcatgagattatcaaaaaggatcttcacctagatccttttaaattaaaaatgaagttttaaatcaatctaaagtatatatgagtaaacttggtctgacagttaccaatgcttaatcagtgaggcacctatctcagcgatctgtctatttcgttcatccatagttgcctgactccccgtcgtgtagataactacgatacgggagggcttaccatctggccccagtgctgcaatgataccgcgagacccacgctcaccggctccagatttatcagcaataaaccagccagccggaagggccgagcgcagaagtggtcctgcaactttatccgcctccatccagtctattaattgttgccgggaagctagagtaagtagttcgccagttaatagtttgcgcaacgttgttgccattgctacaggcatcgtggtgtcacgctcgtcgtttggtatggcttcattcagctccggttcccaacgatcaaggcgagttacatgatcccccatgttgtgcaaaaaagcggttagctccttcggtcctccgatcgttgtcagaagtaagttggccgcagtgttatcactcatggttatggcagcactgcataattctcttactgtcatgccatccgtaagatgcttttctgtgactggtgagtactcaaccaagtcattctgagaatagtgtatgcggcgaccgagttgctcttgcccggcgtcaatacgggataataccgcgccacatagcagaactttaaaagtgctcatcattggaaaacgttcttcggggcgaaaactctcaaggatcttaccgctgttgagatccagttcgatgtaacccactcgtgcacccaactgatcttcagcatcttttactttcaccagcgtttctgggtgagcaaaaacaggaaggcaaaatgccgcaaaaaagggaataagggcgacacggaaatgttgaatactcatactcttcctttttcaatattattgaagcatttatcagggttattgtctcatgagcggatacatatttgaatgtatttagaaaaataaacaaataggggttccgcgcacatttccccgaaaagtgccacctgacgtcgacggatcgggagatcaacttgtttattgcagcttataatggttacaaataaagcaatagcatcacaaatttcacaaataaagcatttttttcactgcattctagttgtggtttgtccaaactcatcaatgtatcttatcatgtctggatcaactggataactcaagctaaccaaaatcatcccaaacttcccaccccataccctattaccactgccaattacctgtggtttcatttactctaaacctgtgattcctctgaattattttcattttaaagaaattgtatttgttaaatatgtactacaaacttagtagt

SEQ ID NO: 20 - protein, 1159 aa, synthetic construct
METPAQLLFLLLLWLPDTTGDIQMTQSPASLSASLEEIVTITCQASQDIGNWLAWYQQKPGKSPQLLIYGATSLADGVPSRFSGSRSGTQFSLKISRVQVEDIGIYYCLQAYNTPWTFGGGTKLELKRGGGGSGGGGSGGGGSEVQLVESGGGLVQPGNSLTLSCVASGFTFSNYGMHWIRQAPKKGLEWIAMIYYDSSKMNYADTVKGRFTISRDNSKNTLYLEMNSLRSEDTAMYYCAVPTSHYVVDVWGQGVSVTVSSGGGGSGGGGSGGGGSAHPGRPRAVPTQCDVPPNSRFDCAPDKAITQEQCEARGCCYIPAKQGLQGAQMGQPWCFFPPSYPSYKLENLSSSEMGYTATLTRTTPTFFPKDILTLRLDVMMETENRLHFTIKDPANRRYEVPLETPRVHSRAPSPLYSVEFSEEPFGVIVHRQLDGRVLLNTTVAPLFFADQFLQLSTSLPSQYITGLAEHLSPLMLSTSWTRITLWNRDLAPTPGANLYGSHPFYLALEDGGSAHGVFLLNSNAMDVVLQPSPALSWRSTGGILDVYIFLGPEPKSVVQQYLDVVGYPFMPPYWGLGFHLCRWGYSSTAITRQVVENMTRAHFPLDVQWNDLDYMDSRRDFTFNKDGFRDFPAMVQELHQGGRRYMMIVDPAISSSGPAGSYRPYDEGLRRGVFITNETGQPLIGKVWPGSTAFPDFTNPTALAWWEDMVAEFHDQVPFDGMWIDMNEPSNFIRGSEDGCPNNELENPPYVPGVVGGTLQAATICASSHQFLSTHYNLHNLYGLTEAIASHRALVKARGTRPFVISRSTFAGHGRYAGHWTGDVWSSWEQLASSVPEILQFNLLGVPLVGADVCGFLGNTSEELCVRWTQLGAFYPFMRNHNSLLSLPQEPYSFSEPAQQAMRKALTLRYALLPHLYTLFHQAHVAGETVARPLFLEFPKDSSTWTVDHQLLWGEALLITPVLQAGKAEVTGYFPLGTWYDLQTVPIEALGSLPPPPAAPREPAIHSEGQWVTLPAPLDTINVHLRAGYIIPLQGPGLTTTESRQQPMALAVALTKGGEARGELFWDDGESLEVLERGAYTQVIFLARNNTIVNELVRVTSEGAGLQLQKVTVLGVATAPQQVLSNGVPVSNFTYSPDTKVLDICVSLLMGEQFLVSWC

SEQ ID NO: 21 - DNA, 3480 bp, synthetic construct
  source 1..3480: mol_type = other DNA
atggaaaccccagcgcagcttctcttcctcctgctactctggctcccagataccaccggagacatccagatgacccagagccccgccagtctgagcgccagcctggaggagatcgtgaccatcacctgccaggcaagccaagacatcggcaactggctggcctggtaccagcagaagcccggcaagagcccccagctgctgatctacggcgccaccagcctggccgacggcgtgcccagccgcttcagcggcagccgcagcggcacccagttcagcctgaagatcagccgcgtgcaggtggaggacatcggcatctactactgcctgcaggcctacaacaccccctggaccttcggcggcggcaccaagctggagctgaagcgcggtggcggagggtctggcggaggaggttccgggggcggtggaagcgaggtgcagctggtggagagcggcggcggcctggtgcagcccggcaacagcctgaccctgagctgcgtggccagcggcttcaccttcagcaactacggcatgcactggatcaggcaggcccccaagaagggcctggagtggatcgccatgatctactacgacagcagcaagatgaactacgccgacaccgtgaagggccgcttcaccatcagccgcgacaacagcaagaacaccctgtacctggagatgaacagcctgcgcagcgaggacaccgccatgtactactgcgccgtgcccaccagccactacgtggtggacgtgtggggacaaggcgtgagcgtgaccgtgagcagcggtggcggagggtctggcggaggaggttccgggggcggtggaagcgcacaccccggccgtcccagagcagtgcccacacagtgcgacgtcccccccaacagccgcttcgattgcgcccctgacaaggccatcacccaggaacagtgcgaggcccgcggctgttgctacatccctgcaaagcaggggctgcagggagcccagatggggcagccctggtgcttcttcccacccagctaccccagctacaagctggagaacctgagctcctctgaaatgggctacacggccaccctgacccgtaccacccccaccttcttccccaaggacatcctgaccctgcggctggacgtgatgatggagactgagaaccgcctccacttcacgatcaaagatccagctaacaggcgctacgaggtgcccttggagaccccgcgtgtccacagccgggcaccgtccccactctacagcgtggagttctccgaggagcccttcggggtgatcgtgcaccggcagctggacggccgcgtgctgctgaacacgacggtggcgcccctgttctttgcggaccagttccttcagctgtccacctcgctgccctcgcagtatatcacaggcctcgccgagcacctcagtcccctgatgctcagcaccagctggaccaggatcaccctgtggaaccgggaccttgcgcccacgcccggtgcgaacctctacgggtctcaccctttctacctggcgctggaggacggcgggtcggcacacggggtgttcctgctaaacagcaatgccatggatgtggtcctgcagccgagccctgcccttagctggaggtcgacaggtgggatcctggatgtctacatcttcctgggcccagagcccaagagcgtggtgcagcagtacctggacgttgtgggatacccgttcatgccgccatactggggcctgggcttccacctgtgccgctggggctactcctccaccgctatcacccgccaggtggtggagaacatgaccagggcccacttccccctggacgtccagtggaacgacctggactacatggactcccggagggacttcacgttcaacaaggatggcttccgggacttcccggccatggtgcaggagctgcaccagggcggccggcgctacatgatgatcgtggatcctgccatcagcagctcgggccctgccgggagctacaggccctacgacgagggtctgcggaggggggttttcatcaccaacgagaccggccagccgctgattgggaaggtatggcccgggtccactgccttccccgacttcaccaaccccacagccctggcctggtgggaggacatggtggctgagttccatgaccaggtgcccttcgacggcatgtggattgacatgaacgagccttccaacttcatcaggggctctgaggacggctgccccaacaatgagctggagaacccaccctacgtgcctggggtggttggggggaccctccaggcggccaccatctgtgcctccagccaccagtttctctccacacactacaacctgcacaacctctacggcctgaccgaagccatcgcctcccacagggcgctggtgaaggctcgggggacacgcccatttgtgatctcccgctcgacctttgctggccacggccgatacgccggccactggacgggggacgtgtggagctcctgggagcagctcgcctcctccgtgccagaaatcctgcagtttaacctgctgggggtgcctctggtcggggccgacgtctgcggcttcctgggcaacacctcagaggagctgtgtgtgcgctggacccagctgggggccttctaccccttcatgcggaaccacaacagcctgctcagtctgccccaggagccgtacagcttcagcgagccggcccagcaggccatgaggaaggccctcaccctgcgctacgcactcctcccccacctctacacactgttccaccaggcccacgtcgcgggggagaccgtggcccggcccctcttcctggagttccccaaggactctagcacctggactgtggaccaccagctcctgtggggggaggccctgctcatcaccccagtgctccaggccgggaaggccgaagtgactggctacttccccttgggcacatggtacgacctgcagacggtgccaatagaggcccttggcagcctcccacccccacctgcagctccccgtgagccagccatccacagcgaggggcagtgggtgacgctgccggcccccctggacaccatcaacgtccacctccgggctgggtacatcatccccctgcagggccctggcctcacaaccacagagtcccgccagcagcccatggccctggctgtggccctgaccaagggtggggaggcccgaggggagctgttctgggacgatggagagagcctggaagtgctggagcgaggggcctacacacaggtcatcttcctggccaggaataacacgatcgtgaatgagctggtacgtgtgaccagtgagggagctggcctgcagctgcagaaggtgactgtcctgggcgtggccacggcgccccagcaggtcctctccaacggtgtccctgtctccaacttcacctacagccccgacaccaaggtcctggacatctgtgtctcgctgttgatgggagagcagtttctcgtcagctggtgttag

SEQ ID NO: 22 - DNA, 9945 bp, synthetic construct
  source 1..9945: mol_type = other DNA
gaattctaatagtaatcaattacggggtcattagttcatagcccatatatggagttccgcgttacataacttacggtaaatggcccgcctggctgaccgcccaacgacccccgcccattgacgtcaataatgacgtatgttcccatagtaacgccaatagggactttccattgacgtcaatgggtggagtatttacggtaaactgcccacttggcagtacatcaagtgtatcatatgccaagtacgccccctattgacgtcaatgacggtaaatggcccgcctggcattatgcccagtacatgaccttatgggactttcctacttggcagtacatctacgtattagtcatcgctattaccatggtgatgcggttttggcagtacatcaatgggcgtggatagcggtttgactcacggggatttccaagtctccaccccattgacgtcaatgggagtttgttttggcaccaaaatcaacgggactttccaaaatgtcgtaacaactccgccccattgacgcaaatgggcggtaggcgtgtacggtgggaggtctatataagcagagctggtttagtgaaccgggtctctctggttagaccagatctgagcctgggagctctctggctaactagggaacccactgcttaagcctcaataaagcttgccttgagtgcttcaagtagtgtgtgcccgtctgttgtgtgactctggtaactagagatccctcagacccttttagtcagtgtggaaaatctctagcagtggcgcccgaacagggacttgaaagcgaaagggaaaccagaggagctctctcgacgcaggactcggcttgctgaagcgcgcacggcaagaggcgaggggcggcgactggtgagtacgccaaaaattttgactagcggaggctagaaggagagagatgggtgcgagagcgtcagtattaagcgggggagaattagatcgcgatgggaaaaaattcggttaaggccagggggaaagaaaaaatataaattaaaacatatagtatgggcaagcagggagctagaacgattcgcagttaatcctggcctgttagaaacatcagaaggctgtagacaaatacgccgctgatcttcagacctggaggaggagatatgagggacaattggagaagtgaattatataaatataaagtagtaaaaattgaaccattaggagtagcacccaccaaggcaaagagaagagtggtgcagagagaaaaaagagcagtgggaataggagctttgttccttgggttcttgggagcagcaggaagcactatgggcgcagcgtcaatgacgctgacggtacaggccagacaattattgtctggtatagtgcagcagcagaacaatttgctgagggctattgaggcgcaacagcatctgttgcaactcacagtctggggcatcaagcagctccaggcaagaatcctggctgtggaaagatacctaaaggatcaacagctcctggggatttggggttgctctggaaaactcatttgcaccactgctgtgccttggaatgctagttggagtaataaatctctggaacagatttggaatcacacgacctggatggagtgggacagagaaattaacaattacacaagcttaatacactccttaattgaagaatcgcaaaaccagcaagaaaagaatgaacaagaattattggaattagataaatgggcaagtttgtggaattggtttaacataacaaattggctgtggtatataaaattattcataatgatagtaggaggcttggtaggtttaagaatagtttttgctgtactttctatagtgaatagagttaggcagggatattcaccattatcgtttcagacccacctcccaaccccgaggggacccgacaggcccgaaggaatagaagaagaaggtggagagagagacagagacagatccattcgattagtgaacggatctcgacggtatcgcctttaaaagaaaaggggggattggggggtacagtgcaggggaaagaatagtagacataatagcaacagacatacaaactaaagaattacaaaaacaaattacaaaaattcaaaattttcgggtttattacagggacagcagagatccagtttatcgatttaaatacgcgtgggaatgaaagaccccacctgtaggtttggcaagctaggatcaaggtcaggaacagagaaacaggagaatatgggccaaacaggatatctgtggtaagcagttcctgccccgctcagggccaagaacagttggaacaggagaatatgggccaaacaggatatctgtggtaagcagttcctgccccgctcagggccaagaacagatggtccccagatgcggtcccgccctcagcagtttctagagaaccatcagatgtttccagggtgccccaaggacctgaaatgaccctgtgccttatttgaactaaccaatcagttcgcttctcgcttctgttcgcgcgcttctgctccccgagctctatataagcagagctggtttagtgaaccgtcagatcggatccgcggccgcgccgccaccatggaaaccccagcgcagcttctcttcctcctgctactctggctcccagataccaccggagacatccagatgacccagagccccgccagtctgagcgccagcctggaggagatcgtgaccatcacctgccaggcaagccaagacatcggcaactggctggcctggtaccagcagaagcccggcaagagcccccagctgctgatctacggcgccaccagcctggccgacggcgtgcccagccgcttcagcggcagccgcagcggcacccagttcagcctgaagatcagccgcgtgcaggtggaggacatcggcatctactactgcctgcaggcctacaacaccccctggaccttcggcggcggcaccaagctggagctgaagcgcggtggcggagggtctggcggaggaggttccgggggcggtggaagcgaggtgcagctggtggagagcggcggcggcctggtgcagcccggcaacagcctgaccctgagctgcgtggccagcggcttcaccttcagcaactacggcatgcactggatcaggcaggcccccaagaagggcctggagtggatcgccatgatctactacgacagcagcaagatgaactacgccgacaccgtgaagggccgcttcaccatcagccgcgacaacagcaagaacaccctgtacctggagatgaacagcctgcgcagcgaggacaccgccatgtactactgcgccgtgcccaccagccactacgtggtggacgtgtggggacaaggcgtgagcgtgaccgtgagcagcggtggcggagggtctggcggaggaggttccgggggcggtggaagcgcacaccccggccgtcccagagcagtgcccacacagtgcgacgtcccccccaacagccgcttcgattgcgcccctgacaaggccatcacccaggaacagtgcgaggcccgcggctgttgctacatccctgcaaagcaggggctgcagggagcccagatggggcagccctggtgcttcttcccacccagctaccccagctacaagctggagaacctgagctcctctgaaatgggctacacggccaccctgacccgtaccacccccaccttcttccccaaggacatcctgaccctgcggctggacgtgatgatggagactgagaaccgcctccacttcacgatcaaagatccagctaacaggcgctacgaggtgcccttggagaccccgcgtgtccacagccgggcaccgtccccactctacagcgtggagttctccgaggagcccttcggggtgatcgtgcaccggcagctggacggccgcgtgctgctgaacacgacggtggcgcccctgttctttgcggaccagttccttcagctgtccacctcgctgccctcgcagtatatcacaggcctcgccgagcacctcagtcccctgatgctcagcaccagctggaccaggatcaccctgtggaaccgggaccttgcgcccacgcccggtgcgaacctctacgggtctcaccctttctacctggcgctggaggacggcgggtcggcacacggggtgttcctgctaaacagcaatgccatggatgtggtcctgcagccgagccctgcccttagctggaggtcgacaggtgggatcctggatgtctacatcttcctgggcccagagcccaagagcgtggtgcagcagtacctggacgttgtgggatacccgttcatgccgccatactggggcctgggcttccacctgtgccgctggggctactcctccaccgctatcacccgccaggtggtggagaacatgaccagggcccacttccccctggacgtccagtggaacgacctggactacatggactcccggagggacttcacgttcaacaaggatggcttccgggacttcccggccatggtgcaggagctgcaccagggcggccggcgctacatgatgatcgtggatcctgccatcagcagctcgggccctgccgggagctacaggccctacgacgagggtctgcggaggggggttttcatcaccaacgagaccggccagccgctgattgggaaggtatggcccgggtccactgccttccccgacttcaccaaccccacagccctggcctggtgggaggacatggtggctgagttccatgaccaggtgcccttcgacggcatgtggattgacatgaacgagccttccaacttcatcaggggctctgaggacggctgccccaacaatgagctggagaacccaccctacgtgcctggggtggttggggggaccctccaggcggccaccatctgtgcctccagccaccagtttctctccacacactacaacctgcacaacctctacggcctgaccgaagccatcgcctcccacagggcgctggtgaaggctcgggggacacgcccatttgtgatctcccgctcgacctttgctggccacggccgatacgccggccactggacgggggacgtgtggagctcctgggagcagctcgcctcctccgtgccagaaatcctgcagtttaacctgctgggggtgcctctggtcggggccgacgtctgcggcttcctgggcaacacctcagaggagctgtgtgtgcgctggacccagctgggggccttctaccccttcatgcggaaccacaacagcctgctcagtctgccccaggagccgtacagcttcagcgagccggcccagcaggccatgaggaaggccctcaccctgcgctacgcactcctcccccacctctacacactgttccaccaggcccacgtcgcgggggagaccgtggcccggcccctcttcctggagttccccaaggactctagcacctggactgtggaccaccagctcctgtggggggaggccctgctcatcaccccagtgctccaggccgggaaggccgaagtgactggctacttccccttgggcacatggtacgacctgcagacggtgccaatagaggcccttggcagcctcccacccccacctgcagctccccgtgagccagccatccacagcgaggggcagtgggtgacgctgccggcccccctggacaccatcaacgtccacctccgggctgggtacatcatccccctgcagggccctggcctcacaaccacagagtcccgccagcagcccatggccctggctgtggccctgaccaagggtggggaggcccgaggggagctgttctgggacgatggagagagcctggaagtgctggagcgaggggcctacacacaggtcatcttcctggccaggaataacacgatcgtgaatgagctggtacgtgtgaccagtgagggagctggcctgcagctgcagaaggtgactgtcctgggcgtggccacggcgccccagcaggtcctctccaacggtgtccctgtctccaacttcacctacagccccgacaccaaggtcctggacatctgtgtctcgctgttgatgggagagcagtttctcgtcagctggtgttagctcgagcctgcaggcgcgtctggaacaatcaacctctggattacaaaatttgtgaaagattgactggtattcttaactatgttgctccttttacgctatgtggatacgctgctttaatgcctttgtatcatgctattgcttcccgtatggctttcattttctcctccttgtataaatcctggttgctgtctctttatgaggagttgtggcccgttgtcaggcaacgtggcgtggtgtgcactgtgtttgctgacgcaacccccactggttggggcattgccaccacctgtcagctcctttccgggactttcgctttccccctccctattgccacggcggaactcatcgccgcctgccttgcccgctgctggacaggggctcggctgttgggcactgacaattccgtggtgttgtcggggaagctgacgtcctttccatggctagctcgcctgtgttgccacctggattctgcgcgggacgtccttctgctacgtcccttcggccctcaatccagcggaccttccttcccgcggcctgctgccggctctgcggcctcttccgcgtcttcgccttcgccctcagacgagtcggatctccctttgggccgcctccccgcctggaattaattctgcagtcgagacctagaaaaacatggagcaatcacaagtagcaatacagcagctaccaatgctgattgtgcctggctagaagcacaagaggaggaggaggtgggttttccagtcacacctcaggtacctttaagaccaatgacttacaaggcagctgtagatcttagccactttttaaaagaaaagaggggactggaagggctaattcactcccaacgaagacaagattctagagggacagcccccccccaaagcccccagggatgtaattacgtccctcccccgctagggggcagcagcgagccgcccggggctccgctccggtccggcgctccccccgcatccccgagccggcagcgtgcggggacagcccgggcacggggaaggtggcacgggatcgctttcctctgaacgcttctcgctgctctttgagcctgcagacacctggggggatacggggaaaaagcttctgctttttgcttgtactgggtctctctggttagaccagatctgagcctgggagctctctggctaactagggaacccactgcttaagcctcaataaagcttgccttgagtgcttcaagtagtgtgtgcccgtctgttgtgtgactctggtaactagagatccctcagacccttttagtcagtgtggaaaatctctagcagtagtagttcatgtcatcttattattcagtatttataacttgcaaagaaatgaatatcagagagtgagaggccttgacattgctagcgttttaccgtcgacctctagctagagcttggcgtaatcatggtcatagctgtttcctgtgtgaaattgttatccgctcacaattccacacaacatacgagccggaagcataaagtgtaaagcctggggtgcctaatgagtgagctaactcacattaattgcgttgcgctcactgcccgctttccagtcgggaaacctgtcgtgccagctgcattaatgaatcggccaacgcgcggggagaggcggtttgcgtattgggcgctcttccgcttcctcgctcactgactcgctgcgctcggtcgttcggctgcggcgagcggtatcagctcactcaaaggcggtaatacggttatccacagaatcaggggataacgcaggaaagaacatgtgagcaaaaggccagcaaaaggccaggaaccgtaaaaaggccgcgttgctggcgtttttccataggctccgcccccctgacgagcatcacaaaaatcgacgctcaagtcagaggtggcgaaacccgacaggactataaagataccaggcgtttccccctggaagctccctcgtgcgctctcctgttccgaccctgccgcttaccggatacctgtccgcctttctcccttcgggaagcgtggcgctttctcatagctcacgctgtaggtatctcagttcggtgtaggtcgttcgctccaagctgggctgtgtgcacgaaccccccgttcagcccgaccgctgcgccttatccggtaactatcgtcttgagtccaacccggtaagacacgacttatcgccactggcagcagccactggtaacaggattagcagagcgaggtatgtaggcggtgctacagagttcttgaagtggtggcctaactacggctacactagaagaacagtatttggtatctgcgctctgctgaagccagttaccttcggaaaaagagttggtagctcttgatccggcaaacaaaccaccgctggtagcggtggtttttttgtttgcaagcagcagattacgcgcagaaaaaaaggatctcaagaagatcctttgatcttttctacggggtctgacgctcagtggaacgaaaactcacgttaagggattttggtcatgagattatcaaaaaggatcttcacctagatccttttaaattaaaaatgaagttttaaatcaatctaaagtatatatgagtaaacttggtctgacagttaccaatgcttaatcagtgaggcacctatctcagcgatctgtctatttcgttcatccatagttgcctgactccccgtcgtgtagataactacgatacgggagggcttaccatctggccccagtgctgcaatgataccgcgagacccacgctcaccggctccagatttatcagcaataaaccagccagccggaagggccgagcgcagaagtggtcctgcaactttatccgcctccatccagtctattaattgttgccgggaagctagagtaagtagttcgccagttaatagtttgcgcaacgttgttgccattgctacaggcatcgtggtgtcacgctcgtcgtttggtatggcttcattcagctccggttcccaacgatcaaggcgagttacatgatcccccatgttgtgcaaaaaagcggttagctccttcggtcctccgatcgttgtcagaagtaagttggccgcagtgttatcactcatggttatggcagcactgcataattctcttactgtcatgccatccgtaagatgcttttctgtgactggtgagtactcaaccaagtcattctgagaatagtgtatgcggcgaccgagttgctcttgcccggcgtcaatacgggataataccgcgccacatagcagaactttaaaagtgctcatcattggaaaacgttcttcggggcgaaaactctcaaggatcttaccgctgttgagatccagttcgatgtaacccactcgtgcacccaactgatcttcagcatcttttactttcaccagcgtttctgggtgagcaaaaacaggaaggcaaaatgccgcaaaaaagggaataagggcgacacggaaatgttgaatactcatactcttcctttttcaatattattgaagcatttatcagggttattgtctcatgagcggatacatatttgaatgtatttagaaaaataaacaaataggggttccgcgcacatttccccgaaaagtgccacctgacgtcgacggatcgggagatcaacttgtttattgcagcttataatggttacaaataaagcaatagcatcacaaatttcacaaataaagcatttttttcactgcattctagttgtggtttgtccaaactcatcaatgtatcttatcatgtctggatcaactggataactcaagctaaccaaaatcatcccaaacttcccaccccataccctattaccactgccaattacctgtggtttcatttactctaaacctgtgattcctctgaattattttcattttaaagaaattgtatttgttaaatatgtactacaaacttagtagt

SEQ ID NO: 23 - protein, 677 aa, synthetic construct
MPGFLVRILPLLLVLLLLGPTRGLRNATQRMFEIDYSRDSFLKDGQPFRYISGSIHYSRVPRFYWKDRLLKMKMAGLNAIQTYVPWNFHEPWPGQYQFSEDHDVEYFLRLAHELGLLVILRPGPYICAEWEMGGLPAWLLEKESILLRSSDPDYLAAVDKWLGVLLPKMKPLLYQNGGPVITVQVENEYGSYFACDFDYLRFLQKRFRHHLGDDVVLFTTDGAHKTFLKCGALQGLYTTVDFGTGSNITDAFLSQRKCEPKGPLINSEFYTGWLDHWGQPHSTIKTEAVASSLYDILARGASVNLYMFIGGTNFAYWNGANSPYAAQPTSYDYDAPLSEAGDLTEKYFALRNIIQKFEKVPEGPIPPSTPKFAYGKVTLEKLKTVGAALDILCPSGPIKSLYPLTFIQVKQHYGFVLYRTTLPQDCSNPAPLSSPLNGVHDRAYVAVDGIPQGVLERNNVITLNITGKAGATLDLLVENMGRVNYGAYINDFKGLVSNLTLSSNILTDWTIFPLDTEDAVRSHLGGWGHRDSGHHDEAWAHNSSNYTLPAFYMGNFSIPSGIPDLPQDTFIQFPGWTKGQVWINGFNLGRYWPARGPQLTLFVPQHILMTSAPNTITVLELEWAPCSSDDPELCAVTFVDRPVIGSSVTYDHPSKPVEKRLMPPPPQKNKDSWLDHV

SEQ ID NO: 24 - DNA, 2034 bp, synthetic construct
  source 1..2034: mol_type = other DNA
atgccggggttcctggttcgcatcctccctctgctgctggttctgctgcttctgggccctacgcgcggcttgcgcaatgccacccagaggatgttcgaaattgattactcccgggatagcttcctcaaagacggccagccttttaggtacatctccggctccattcactattcccgggtgcctcgtttttactggaaagaccggctgctgaagatgaagatggccggactgaacgctatccagacctacgtcccttggaactttcatgagccttggcccggccagtaccaatttagcgaggaccacgacgtcgagtactttttacggctggcccacgaactcggactcctcgtgattctgaggcccggcccctacatttgcgccgagtgggagatgggaggtttacccgcttggctgctggagaaggagtccatcttattacggagcagcgatcccgattatttagccgccgtggacaaatggctgggagttttactccccaagatgaaacctttactgtaccagaatggcggccccgttatcaccgtccaagttgagaatgagtatggctcctatttcgcttgcgacttcgactatttacggtttttacagaagaggtttcgtcaccacctcggagacgatgtcgtcctcttcaccaccgatggagcccataagacctttttaaagtgtggcgccctccaaggtttatataccaccgtggatttcggcactggtagcaacatcacagatgcctttctctcccagcggaagtgcgaacctaagggccctttaatcaattccgagttctacaccggctggctcgaccactggggccagcctcactccaccatcaagacagaagccgtggccagctctttatacgacatcctcgctcggggcgcctccgtcaatttatacatgtttatcggcggcaccaacttcgcctattggaacggcgctaactccccctacgccgctcagcccacaagctatgactatgatgcccctctgtccgaagccggagatttaaccgagaagtacttcgccctccggaacatcattcagaagttcgagaaggtgcccgagggacccatccctcccagcacccccaagttcgcttacggaaaagtcaccctcgaaaaactgaagaccgtgggcgccgctttagatattctgtgccccagcggccctattaagtctttataccccctcacctttattcaagttaagcagcattacggctttgttttataccggaccactttaccccaagattgtagcaaccccgctcctctgagcagccctttaaacggcgtccatgatcgggcttatgtggctgtcgacggcattccccaaggtgtgctcgaacggaacaacgtgatcactttaaatatcaccggcaaagctggcgctacactggatctgctggtcgaaaacatgggccgggtgaactacggcgcctacattaacgatttcaagggtttagtgtccaatttaacactcagctccaacattctcaccgactggaccatcttccctttagacaccgaggatgctgtgaggagccatttaggcggatggggccatcgggacagcggacatcacgacgaggcttgggctcacaatagctccaactacacactgcccgctttctacatgggcaacttcagcatccctagcggaattcccgatctgcctcaagataccttcatccaattccccggctggaccaagggccaagtttggatcaacggctttaatttaggccggtactggcccgctcgtggacctcagctgacactgttcgtgcctcaacacattttaatgacctccgctcctaacacaatcaccgtgctggagctggagtgggctccttgtagctccgacgatcccgagctgtgcgccgtcaccttcgtcgatcgtcccgtcatcggctcctccgtgacatacgaccaccccagcaagcccgttgagaagcggctgatgcctcctcctcctcagaagaacaaggactcttggctggaccacgtgtaa

SEQ ID NO: 25 - DNA, 8488 bp, synthetic construct
  source 1..8488: mol_type = other DNA
gaattctaatagtaatcaattacggggtcattagttcatagcccatatatggagttccgcgttacataacttacggtaaatggcccgcctggctgaccgcccaacgacccccgcccattgacgtcaataatgacgtatgttcccatagtaacgccaatagggactttccattgacgtcaatgggtggagtatttacggtaaactgcccacttggcagtacatcaagtgtatcatatgccaagtacgccccctattgacgtcaatgacggtaaatggcccgcctggcattatgcccagtacatgaccttatgggactttcctacttggcagtacatctacgtattagtcatcgctattaccatggtgatgcggttttggcagtacatcaatgggcgtggatagcggtttgactcacggggatttccaagtctccaccccattgacgtcaatgggagtttgttttggcaccaaaatcaacgggactttccaaaatgtcgtaacaactccgccccattgacgcaaatgggcggtaggcgtgtacggtgggaggtctatataagcagagctggtttagtgaaccgggtctctctggttagaccagatctgagcctgggagctctctggctaactagggaacccactgcttaagcctcaataaagcttgccttgagtgcttcaagtagtgtgtgcccgtctgttgtgtgactctggtaactagagatccctcagacccttttagtcagtgtggaaaatctctagcagtggcgcccgaacagggacttgaaagcgaaagggaaaccagaggagctctctcgacgcaggactcggcttgctgaagcgcgcacggcaagaggcgaggggcggcgactggtgagtacgccaaaaattttgactagcggaggctagaaggagagagatgggtgcgagagcgtcagtattaagcgggggagaattagatcgcgatgggaaaaaattcggttaaggccagggggaaagaaaaaatataaattaaaacatatagtatgggcaagcagggagctagaacgattcgcagttaatcctggcctgttagaaacatcagaaggctgtagacaaatacgccgctgatcttcagacctggaggaggagatatgagggacaattggagaagtgaattatataaatataaagtagtaaaaattgaaccattaggagtagcacccaccaaggcaaagagaagagtggtgcagagagaaaaaagagcagtgggaataggagctttgttccttgggttcttgggagcagcaggaagcactatgggcgcagcgtcaatgacgctgacggtacaggccagacaattattgtctggtatagtgcagcagcagaacaatttgctgagggctattgaggcgcaacagcatctgttgcaactcacagtctggggcatcaagcagctccaggcaagaatcctggctgtggaaagatacctaaaggatcaacagctcctggggatttggggttgctctggaaaactcatttgcaccactgctgtgccttggaatgctagttggagtaataaatctctggaacagatttggaatcacacgacctggatggagtgggacagagaaattaacaattacacaagcttaatacactccttaattgaagaatcgcaaaaccagcaagaaaagaatgaacaagaattattggaattagataaatgggcaagtttgtggaattggtttaacataacaaattggctgtggtatataaaattattcataatgatagtaggaggcttggtaggtttaagaatagtttttgctgtactttctatagtgaatagagttaggcagggatattcaccattatcgtttcagacccacctcccaaccccgaggggacccgacaggcccgaaggaatagaagaagaaggtggagagagagacagagacagatccattcgattagtgaacggatctcgacggtatcgcctttaaaagaaaaggggggattggggggtacagtgcaggggaaagaatagtagacataatagcaacagacatacaaactaaagaattacaaaaacaaattacaaaaattcaaaattttcgggtttattacagggacagcagagatccagtttatcgatttaaatacgcgtgggaatgaaagaccccacctgtaggtttggcaagctaggatcaaggtcaggaacagagaaacaggagaatatgggccaaacaggatatctgtggtaagcagttcctgccccgctcagggccaagaacagttggaacaggagaatatgggccaaacaggatatctgtggtaagcagttcctgccccgctcagggccaagaacagatggtccccagatgcggtcccgccctcagcagtttctagagaaccatcagatgtttccagggtgccccaaggacctgaaatgaccctgtgccttatttgaactaaccaatcagttcgcttctcgcttctgttcgcgcgcttctgctccccgagctctatataagcagagctggtttagtgaaccgtcagatcggatccgccaccatgccggggttcctggttcgcatcctccctctgctgctggttctgctgcttctgggccctacgcgcggcttgcgcaatgccacccagaggatgttcgaaattgattactcccgggatagcttcctcaaagacggccagccttttaggtacatctccggctccattcactattcccgggtgcctcgtttttactggaaagaccggctgctgaagatgaagatggccggactgaacgctatccagacctacgtcccttggaactttcatgagccttggcccggccagtaccaatttagcgaggaccacgacgtcgagtactttttacggctggcccacgaactcggactcctcgtgattctgaggcccggcccctacatttgcgccgagtgggagatgggaggtttacccgcttggctgctggagaaggagtccatcttattacggagcagcgatcccgattatttagccgccgtggacaaatggctgggagttttactccccaagatgaaacctttactgtaccagaatggcggccccgttatcaccgtccaagttgagaatgagtatggctcctatttcgcttgcgacttcgactatttacggtttttacagaagaggtttcgtcaccacctcggagacgatgtcgtcctcttcaccaccgatggagcccataagacctttttaaagtgtggcgccctccaaggtttatataccaccgtggatttcggcactggtagcaacatcacagatgcctttctctcccagcggaagtgcgaacctaagggccctttaatcaattccgagttctacaccggctggctcgaccactggggccagcctcactccaccatcaagacagaagccgtggccagctctttatacgacatcctcgctcggggcgcctccgtcaatttatacatgtttatcggcggcaccaacttcgcctattggaacggcgctaactccccctacgccgctcagcccacaagctatgactatgatgcccctctgtccgaagccggagatttaaccgagaagtacttcgccctccggaacatcattcagaagttcgagaaggtgcccgagggacccatccctcccagcacccccaagttcgcttacggaaaagtcaccctcgaaaaactgaagaccgtgggcgccgctttagatattctgtgccccagcggccctattaagtctttataccccctcacctttattcaagttaagcagcattacggctttgttttataccggaccactttaccccaagattgtagcaaccccgctcctctgagcagccctttaaacggcgtccatgatcgggcttatgtggctgtcgacggcattccccaaggtgtgctcgaacggaacaacgtgatcactttaaatatcaccggcaaagctggcgctacactggatctgctggtcgaaaacatgggccgggtgaactacggcgcctacattaacgatttcaagggtttagtgtccaatttaacactcagctccaacattctcaccgactggaccatcttccctttagacaccgaggatgctgtgaggagccatttaggcggatggggccatcgggacagcggacatcacgacgaggcttgggctcacaatagctccaactacacactgcccgctttctacatgggcaacttcagcatccctagcggaattcccgatctgcctcaagataccttcatccaattccccggctggaccaagggccaagtttggatcaacggctttaatttaggccggtactggcccgctcgtggacctcagctgacactgttcgtgcctcaacacattttaatgacctccgctcctaacacaatcaccgtgctggagctggagtgggctccttgtagctccgacgatcccgagctgtgcgccgtcaccttcgtcgatcgtcccgtcatcggctcctccgtgacatacgaccaccccagcaagcccgttgagaagcggctgatgcctcctcctcctcagaagaacaaggactcttggctggaccacgtgtaactcgagcctgcaggcgcgtctggaacaatcaacctctggattacaaaatttgtgaaagattgactggtattcttaactatgttgctccttttacgctatgtggatacgctgctttaatgcctttgtatcatgctattgcttcccgtatggctttcattttctcctccttgtataaatcctggttgctgtctctttatgaggagttgtggcccgttgtcaggcaacgtggcgtggtgtgcactgtgtttgctgacgcaacccccactggttggggcattgccaccacctgtcagctcctttccgggactttcgctttccccctccctattgccacggcggaactcatcgccgcctgccttgcccgctgctggacaggggctcggctgttgggcactgacaattccgtggtgttgtcggggaagctgacgtcctttccatggctagctcgcctgtgttgccacctggattctgcgcgggacgtccttctgctacgtcccttcggccctcaatccagcggaccttccttcccgcggcctgctgccggctctgcggcctcttccgcgtcttcgccttcgccctcagacgagtcggatctccctttgggccgcctccccgcctggaattaattctgcagtcgagacctagaaaaacatggagcaatcacaagtagcaatacagcagctaccaatgctgattgtgcctggctagaagcacaagaggaggaggaggtgggttttccagtcacacctcaggtacctttaagaccaatgacttacaaggcagctgtagatcttagccactttttaaaagaaaagaggggactggaagggctaattcactcccaacgaagacaagattctagagggacagcccccccccaaagcccccagggatgtaattacgtccctcccccgctagggggcagcagcgagccgcccggggctccgctccggtccggcgctccccccgcatccccgagccggcagcgtgcggggacagcccgggcacggggaaggtggcacgggatcgctttcctctgaacgcttctcgctgctctttgagcctgcagacacctggggggatacggggaaaaagcttctgctttttgcttgtactgggtctctctggttagaccagatctgagcctgggagctctctggctaactagggaacccactgcttaagcctcaataaagcttgccttgagtgcttcaagtagtgtgtgcccgtctgttgtgtgactctggtaactagagatccctcagacccttttagtcagtgtggaaaatctctagcagtagtagttcatgtcatcttattattcagtatttataacttgcaaagaaatgaatatcagagagtgagaggccttgacattgctagcgttttaccgtcgacctctagctagagcttggcgtaatcatggtcatagctgtttcctgtgtgaaattgttatccgctcacaattccacacaacatacgagccggaagcataaagtgtaaagcctggggtgcctaatgagtgagctaactcacattaattgcgttgcgctcactgcccgctttccagtcgggaaacctgtcgtgccagctgcattaatgaatcggccaacgcgcggggagaggcggtttgcgtattgggcgctcttccgcttcctcgctcactgactcgctgcgctcggtcgttcggctgcggcgagcggtatcagctcactcaaaggcggtaatacggttatccacagaatcaggggataacgcaggaaagaacatgtgagcaaaaggccagcaaaaggccaggaaccgtaaaaaggccgcgttgctggcgtttttccataggctccgcccccctgacgagcatcacaaaaatcgacgctcaagtcagaggtggcgaaacccgacaggactataaagataccaggcgtttccccctggaagctccctcgtgcgctctcctgttccgaccctgccgcttaccggatacctgtccgcctttctcccttcgggaagcgtggcgctttctcatagctcacgctgtaggtatctcagttcggtgtaggtcgttcgctccaagctgggctgtgtgcacgaaccccccgttcagcccgaccgctgcgccttatccggtaactatcgtcttgagtccaacccggtaagacacgacttatcgccactggcagcagccactggtaacaggattagcagagcgaggtatgtaggcggtgctacagagttcttgaagtggtggcctaactacggctacactagaagaacagtatttggtatctgcgctctgctgaagccagttaccttcggaaaaagagttggtagctcttgatccggcaaacaaaccaccgctggtagcggtggtttttttgtttgcaagcagcagattacgcgcagaaaaaaaggatctcaagaagatcctttgatcttttctacggggtctgacgctcagtggaacgaaaactcacgttaagggattttggtcatgagattatcaaaaaggatcttcacctagatccttttaaattaaaaatgaagttttaaatcaatctaaagtatatatgagtaaacttggtctgacagttaccaatgcttaatcagtgaggcacctatctcagcgatctgtctatttcgttcatccatagttgcctgactccccgtcgtgtagataactacgatacgggagggcttaccatctggccccagtgctgcaatgataccgcgagacccacgctcaccggctccagatttatcagcaataaaccagccagccggaagggccgagcgcagaagtggtcctgcaactttatccgcctccatccagtctattaattgttgccgggaagctagagtaagtagttcgccagttaatagtttgcgcaacgttgttgccattgctacaggcatcgtggtgtcacgctcgtcgtttggtatggcttcattcagctccggttcccaacgatcaaggcgagttacatgatcccccatgttgtgcaaaaaagcggttagctccttcggtcctccgatcgttgtcagaagtaagttggccgcagtgttatcactcatggttatggcagcactgcataattctcttactgtcatgccatccgtaagatgcttttctgtgactggtgagtactcaaccaagtcattctgagaatagtgtatgcggcgaccgagttgctcttgcccggcgtcaatacgggataataccgcgccacatagcagaactttaaaagtgctcatcattggaaaacgttcttcggggcgaaaactctcaaggatcttaccgctgttgagatccagttcgatgtaacccactcgtgcacccaactgatcttcagcatcttttactttcaccagcgtttctgggtgagcaaaaacaggaaggcaaaatgccgcaaaaaagggaataagggcgacacggaaatgttgaatactcatactcttcctttttcaatattattgaagcatttatcagggttattgtctcatgagcggatacatatttgaatgtatttagaaaaataaacaaataggggttccgcgcacatttccccgaaaagtgccacctgacgtcgacggatcgggagatcaacttgtttattgcagcttataatggttacaaataaagcaatagcatcacaaatttcacaaataaagcatttttttcactgcattctagttgtggtttgtccaaactcatcaatgtatcttatcatgtctggatcaactggataactcaagctaaccaaaatcatcccaaacttcccaccccataccctattaccactgccaattacctgtggtttcatttactctaaacctgtgattcctctgaattattttcattttaaagaaattgtatttgttaaatatgtactacaaacttagtagt

SEQ ID NO: 26 - protein, 924 aa, synthetic construct
MGWSCIILFLVATATGVHSEVQLVESGGGLVQPGNSLTLSCVASGFTFSNYGMHWIRQAPKKGLEWIAMIYYDSSKMNYADTVKGRFTISRDNSKNTLYLEMNSLRSEDTAMYYCAVPTSHYVVDVWGQGVSVTVSSGGGGSGGGGSGGGGSDIQMTQSPASLSASLEEIVTITCQASQDIGNWLAWYQQKPGKSPQLLIYGATSLADGVPSRFSGSRSGTQFSLKISRVQVEDIGIYYCLQAYNTPWTFGGGTKLELKRGGGGSGGGGSGGGGSQRMFEIDYSRDSFLKDGQPFRYISGSIHYSRVPRFYWKDRLLKMKMAGLNAIQTYVPWNFHEPWPGQYQFSEDHDVEYFLRLAHELGLLVILRPGPYICAEWEMGGLPAWLLEKESILLRSSDPDYLAAVDKWLGVLLPKMKPLLYQNGGPVITVQVENEYGSYFACDFDYLRFLQKRFRHHLGDDVVLFTTDGAHKTFLKCGALQGLYTTVDFGTGSNITDAFLSQRKCEPKGPLINSEFYTGWLDHWGQPHSTIKTEAVASSLYDILARGASVNLYMFIGGTNFAYWNGANSPYAAQPTSYDYDAPLSEAGDLTEKYFALRNIIQKFEKVPEGPIPPSTPKFAYGKVTLEKLKTVGAALDILCPSGPIKSLYPLTFIQVKQHYGFVLYRTTLPQDCSNPAPLSSPLNGVHDRAYVAVDGIPQGVLERNNVITLNITGKAGATLDLLVENMGRVNYGAYINDFKGLVSNLTLSSNILTDWTIFPLDTEDAVRSHLGGWGHRDSGHHDEAWAHNSSNYTLPAFYMGNFSIPSGIPDLPQDTFIQFPGWTKGQVWINGFNLGRYWPARGPQLTLFVPQHILMTSAPNTITVLELEWAPCSSDDPELCAVTFVDRPVIGSSVTYDHPSKPVEKRLMPPPPQKNKDSWLDHV

SEQ ID NO: 27 - DNA, 2775 bp, synthetic construct
  source 1..2775: mol_type = other DNA
atgggctggagctgcattattctgtttctggtggcgaccgcgaccggcgtgcatagcgaggtgcagctggtggagagcggcggcggcctggtgcagcccggcaacagcctgaccctgagctgcgtggccagcggcttcaccttcagcaactacggcatgcactggatcaggcaggcccccaagaagggcctggagtggatcgccatgatctactacgacagcagcaagatgaactacgccgacaccgtgaagggccgcttcaccatcagccgcgacaacagcaagaacaccctgtacctggagatgaacagcctgcgcagcgaggacaccgccatgtactactgcgccgtgcccaccagccactacgtggtggacgtgtggggacaaggcgtgagcgtgaccgtgagcagcggtggcggagggtctggcggaggaggttccgggggcggtggaagcgacatccagatgacccagagccccgccagtctgagcgccagcctggaggagatcgtgaccatcacctgccaggcaagccaagacatcggcaactggctggcctggtaccagcagaagcccggcaagagcccccagctgctgatctacggcgccaccagcctggccgacggcgtgcccagccgcttcagcggcagccgcagcggcacccagttcagcctgaagatcagccgcgtgcaggtggaggacatcggcatctactactgcctgcaggcctacaacaccccctggaccttcggcggcggcaccaagctggagctgaagcgcggtggcggagggtctggaggtggcggatcaggcggaggaggatctcagaggatgttcgaaattgattactcccgggatagcttcctcaaagacggccagccttttaggtacatctccggctccattcactattcccgggtgcctcgtttttactggaaagaccggctgctgaagatgaagatggccggactgaacgctatccagacctacgtcccttggaactttcatgagccttggcccggccagtaccaatttagcgaggaccacgacgtcgagtactttttacggctggcccacgaactcggactcctcgtgattctgaggcccggcccctacatttgcgccgagtgggagatgggaggtttacccgcttggctgctggagaaggagtccatcttattacggagcagcgatcccgattatttagccgccgtggacaaatggctgggagttttactccccaagatgaaacctttactgtaccagaatggcggccccgttatcaccgtccaagttgagaatgagtatggctcctatttcgcttgcgacttcgactatttacggtttttacagaagaggtttcgtcaccacctcggagacgatgtcgtcctcttcaccaccgatggagcccataagacctttttaaagtgtggcgccctccaaggtttatataccaccgtggatttcggcactggtagcaacatcacagatgcctttctctcccagcggaagtgcgaacctaagggccctttaatcaattccgagttctacaccggctggctcgaccactggggccagcctcactccaccatcaagacagaagccgtggccagctctttatacgacatcctcgctcggggcgcctccgtcaatttatacatgtttatcggcggcaccaacttcgcctattggaacggcgctaactccccctacgccgctcagcccacaagctatgactatgatgcccctctgtccgaagccggagatttaaccgagaagtacttcgccctccggaacatcattcagaagttcgagaaggtgcccgagggacccatccctcccagcacccccaagttcgcttacggaaaagtcaccctcgaaaaactgaagaccgtgggcgccgctttagatattctgtgccccagcggccctattaagtctttataccccctcacctttattcaagttaagcagcattacggctttgttttataccggaccactttaccccaagattgtagcaaccccgctcctctgagcagccctttaaacggcgtccatgatcgggcttatgtggctgtcgacggcattccccaaggtgtgctcgaacggaacaacgtgatcactttaaatatcaccggcaaagctggcgctacactggatctgctggtcgaaaacatgggccgggtgaactacggcgcctacattaacgatttcaagggtttagtgtccaatttaacactcagctccaacattctcaccgactggaccatcttccctttagacaccgaggatgctgtgaggagccatttaggcggatggggccatcgggacagcggacatcacgacgaggcttgggctcacaatagctccaactacacactgcccgctttctacatgggcaacttcagcatccctagcggaattcccgatctgcctcaagataccttcatccaattccccggctggaccaagggccaagtttggatcaacggctttaatttaggccggtactggcccgctcgtggacctcagctgacactgttcgtgcctcaacacattttaatgacctccgctcctaacacaatcaccgtgctggagctggagtgggctccttgtagctccgacgatcccgagctgtgcgccgtcaccttcgtcgatcgtcccgtcatcggctcctccgtgacatacgaccaccccagcaagcccgttgagaagcggctgatgcctcctcctcctcagaagaacaaggactcttggctggaccacgtgtga

SEQ ID NO: 28 - DNA, 9246 bp, synthetic construct
  source 1..9246: mol_type = other DNA
gaattctaatagtaatcaattacggggtcattagttcatagcccatatatggagttccgcgttacataacttacggtaaatggcccgcctggctgaccgcccaacgacccccgcccattgacgtcaataatgacgtatgttcccatagtaacgccaatagggactttccattgacgtcaatgggtggagtatttacggtaaactgcccacttggcagtacatcaagtgtatcatatgccaagtacgccccctattgacgtcaatgacggtaaatggcccgcctggcattatgcccagtacatgaccttatgggactttcctacttggcagtacatctacgtattagtcatcgctattaccatggtgatgcggttttggcagtacatcaatgggcgtggatagcggtttgactcacggggatttccaagtctccaccccattgacgtcaatgggagtttgttttggcaccaaaatcaacgggactttccaaaatgtcgtaacaactccgccccattgacgcaaatgggcggtaggcgtgtacggtgggaggtctatataagcagagctggtttagtgaaccgggtctctctggttagaccagatctgagcctgggagctctctggctaactagggaacccactgcttaagcctcaataaagcttgccttgagtgcttcaagtagtgtgtgcccgtctgttgtgtgactctggtaactagagatccctcagacccttttagtcagtgtggaaaatctctagcagtggcgcccgaacagggacttgaaagcgaaagggaaaccagaggagctctctcgacgcaggactcggcttgctgaagcgcgcacggcaagaggcgaggggcggcgactggtgagtacgccaaaaattttgactagcggaggctagaaggagagagatgggtgcgagagcgtcagtattaagcgggggagaattagatcgcgatgggaaaaaattcggttaaggccagggggaaagaaaaaatataaattaaaacatatagtatgggcaagcagggagctagaacgattcgcagttaatcctggcctgttagaaacatcagaaggctgtagacaaatacgccgctgatcttcagacctggaggaggagatatgagggacaattggagaagtgaattatataaatataaagtagtaaaaattgaaccattaggagtagcacccaccaaggcaaagagaagagtggtgcagagagaaaaaagagcagtgggaataggagctttgttccttgggttcttgggagcagcaggaagcactatgggcgcagcgtcaatgacgctgacggtacaggccagacaattattgtctggtatagtgcagcagcagaacaatttgctgagggctattgaggcgcaacagcatctgttgcaactcacagtctggggcatcaagcagctccaggcaagaatcctggctgtggaaagatacctaaaggatcaacagctcctggggatttggggttgctctggaaaactcatttgcaccactgctgtgccttggaatgctagttggagtaataaatctctggaacagatttggaatcacacgacctggatggagtgggacagagaaattaacaattacacaagcttaatacactccttaattgaagaatcgcaaaaccagcaagaaaagaatgaacaagaattattggaattagataaatgggcaagtttgtggaattggtttaacataacaaattggctgtggtatataaaattattcataatgatagtaggaggcttggtaggtttaagaatagtttttgctgtactttctatagtgaatagagttaggcagggatattcaccattatcgtttcagacccacctcccaaccccgaggggacccgacaggcccgaaggaatagaagaagaaggtggagagagagacagagacagatccattcgattagtgaacggatctcgacggtatcgcctttaaaagaaaaggggggattggggggtacagtgcaggggaaagaatagtagacataatagcaacagacatacaaactaaagaattacaaaaacaaattacaaaaattcaaaattttcgggtttattacagggacagcagagatccagtttatcgatttaaatacgcgtgggaatgaaagaccccacctgtaggtttggcaagctaggatcaaggtcaggaacagagaaacaggagaatatgggccaaacaggatatctgtggtaagcagttcctgccccgctcagggccaagaacagttggaacaggagaatatgggccaaacaggatatctgtggtaagcagttcctgccccgctcagggccaagaacagatggtccccagatgcggtcccgccctcagcagtttctagagaaccatcagatgtttccagggtgccccaaggacctgaaatgaccctgtgccttatttgaactaaccaatcagttcgcttctcgcttctgttcgcgcgcttctgctccccgagctctatataagcagagctggtttagtgaaccgtcagatcggatccgcggccgcgccgccaccatgggctggagctgcattattctgtttctggtggcgaccgcgaccggcgtgcatagcgaggtgcagctggtggagagcggcggcggcctggtgcagcccggcaacagcctgaccctgagctgcgtggccagcggcttcaccttcagcaactacggcatgcactggatcaggcaggcccccaagaagggcctggagtggatcgccatgatctactacgacagcagcaagatgaactacgccgacaccgtgaagggccgcttcaccatcagccgcgacaacagcaagaacaccctgtacctggagatgaacagcctgcgcagcgaggacaccgccatgtactactgcgccgtgcccaccagccactacgtggtggacgtgtggggacaaggcgtgagcgtgaccgtgagcagcggtggcggagggtctggcggaggaggttccgggggcggtggaagcgacatccagatgacccagagccccgccagtctgagcgccagcctggaggagatcgtgaccatcacctgccaggcaagccaagacatcggcaactggctggcctggtaccagcagaagcccggcaagagcccccagctgctgatctacggcgccaccagcctggccgacggcgtgcccagccgcttcagcggcagccgcagcggcacccagttcagcctgaagatcagccgcgtgcaggtggaggacatcggcatctactactgcctgcaggcctacaacaccccctggaccttcggcggcggcaccaagctggagctgaagcgcggtggcggagggtctggaggtggcggatcaggcggaggaggatctcagaggatgttcgaaattgattactcccgggatagcttcctcaaagacggccagccttttaggtacatctccggctccattcactattcccgggtgcctcgtttttactggaaagaccggctgctgaagatgaagatggccggactgaacgctatccagacctacgtcccttggaactttcatgagccttggcccggccagtaccaatttagcgaggaccacgacgtcgagtactttttacggctggcccacgaactcggactcctcgtgattctgaggcccggcccctacatttgcgccgagtgggagatgggaggtttacccgcttggctgctggagaaggagtccatcttattacggagcagcgatcccgattatttagccgccgtggacaaatggctgggagttttactccccaagatgaaacctttactgtaccagaatggcggccccgttatcaccgtccaagttgagaatgagtatggctcctatttcgcttgcgacttcgactatttacggtttttacagaagaggtttcgtcaccacctcggagacgatgtcgtcctcttcaccaccgatggagcccataagacctttttaaagtgtggcgccctccaaggtttatataccaccgtggatttcggcactggtagcaacatcacagatgcctttctctcccagcggaagtgcgaacctaagggccctttaatcaattccgagttctacaccggctggctcgaccactggggccagcctcactccaccatcaagacagaagccgtggccagctctttatacgacatcctcgctcggggcgcctccgtcaatttatacatgtttatcggcggcaccaacttcgcctattggaacggcgctaactccccctacgccgctcagcccacaagctatgactatgatgcccctctgtccgaagccggagatttaaccgagaagtacttcgccctccggaacatcattcagaagttcgagaaggtgcccgagggacccatccctcccagcacccccaagttcgcttacggaaaagtcaccctcgaaaaactgaagaccgtgggcgccgctttagatattctgtgccccagcggccctattaagtctttataccccctcacctttattcaagttaagcagcattacggctttgttttataccggaccactttaccccaagattgtagcaaccccgctcctctgagcagccctttaaacggcgtccatgatcgggcttatgtggctgtcgacggcattccccaaggtgtgctcgaacggaacaacgtgatcactttaaatatcaccggcaaagctggcgctacactggatctgctggtcgaaaacatgggccgggtgaactacggcgcctacattaacgatttcaagggtttagtgtccaatttaacactcagctccaacattctcaccgactggaccatcttccctttagacaccgaggatgctgtgaggagccatttaggcggatggggccatcgggacagcggacatcacgacgaggcttgggctcacaatagctccaactacacactgcccgctttctacatgggcaacttcagcatccctagcggaattcccgatctgcctcaagataccttcatccaattccccggctggaccaagggccaagtttggatcaacggctttaatttaggccggtactggcccgctcgtggacctcagctgacactgttcgtgcctcaacacattttaatgacctccgctcctaacacaatcaccgtgctggagctggagtgggctccttgtagctccgacgatcccgagctgtgcgccgtcaccttcgtcgatcgtcccgtcatcggctcctccgtgacatacgaccaccccagcaagcccgttgagaagcggctgatgcctcctcctcctcagaagaacaaggactcttggctggaccacgtgtgatgatgactcgagcctgcaggcgcgtctggaacaatcaacctctggattacaaaatttgtgaaagattgactggtattcttaactatgttgctccttttacgctatgtggatacgctgctttaatgcctttgtatcatgctattgcttcccgtatggctttcattttctcctccttgtataaatcctggttgctgtctctttatgaggagttgtggcccgttgtcaggcaacgtggcgtggtgtgcactgtgtttgctgacgcaacccccactggttggggcattgccaccacctgtcagctcctttccgggactttcgctttccccctccctattgccacggcggaactcatcgccgcctgccttgcccgctgctggacaggggctcggctgttgggcactgacaattccgtggtgttgtcggggaagctgacgtcctttccatggctagctcgcctgtgttgccacctggattctgcgcgggacgtccttctgctacgtcccttcggccctcaatccagcggaccttccttcccgcggcctgctgccggctctgcggcctcttccgcgtcttcgccttcgccctcagacgagtcggatctccctttgggccgcctccccgcctggaattaattctgcagtcgagacctagaaaaacatggagcaatcacaagtagcaatacagcagctaccaatgctgattgtgcctggctagaagcacaagaggaggaggaggtgggttttccagtcacacctcaggtacctttaagaccaatgacttacaaggcagctgtagatcttagccactttttaaaagaaaagaggggactggaagggctaattcactcccaacgaagacaagattctagagggacagcccccccccaaagcccccagggatgtaattacgtccctcccccgctagggggcagcagcgagccgcccggggctccgctccggtccggcgctccccccgcatccccgagccggcagcgtgcggggacagcccgggcacggggaaggtggcacgggatcgctttcctctgaacgcttctcgctgctctttgagcctgcagacacctggggggatacggggaaaaagcttctgctttttgcttgtactgggtctctctggttagaccagatctgagcctgggagctctctggctaactagggaacccactgcttaagcctcaataaagcttgccttgagtgcttcaagtagtgtgtgcccgtctgttgtgtgactctggtaactagagatccctcagacccttttagtcagtgtggaaaatctctagcagtagtagttcatgtcatcttattattcagtatttataacttgcaaagaaatgaatatcagagagtgagaggccttgacattgctagcgttttaccgtcgacctctagctagagcttggcgtaatcatggtcatagctgtttcctgtgtgaaattgttatccgctcacaattccacacaacatacgagccggaagcataaagtgtaaagcctggggtgcctaatgagtgagctaactcacattaattgcgttgcgctcactgcccgctttccagtcgggaaacctgtcgtgccagctgcattaatgaatcggccaacgcgcggggagaggcggtttgcgtattgggcgctcttccgcttcctcgctcactgactcgctgcgctcggtcgttcggctgcggcgagcggtatcagctcactcaaaggcggtaatacggttatccacagaatcaggggataacgcaggaaagaacatgtgagcaaaaggccagcaaaaggccaggaaccgtaaaaaggccgcgttgctggcgtttttccataggctccgcccccctgacgagcatcacaaaaatcgacgctcaagtcagaggtggcgaaacccgacaggactataaagataccaggcgtttccccctggaagctccctcgtgcgctctcctgttccgaccctgccgcttaccggatacctgtccgcctttctcccttcgggaagcgtggcgctttctcatagctcacgctgtaggtatctcagttcggtgtaggtcgttcgctccaagctgggctgtgtgcacgaaccccccgttcagcccgaccgctgcgccttatccggtaactatcgtcttgagtccaacccggtaagacacgacttatcgccactggcagcagccactggtaacaggattagcagagcgaggtatgtaggcggtgctacagagttcttgaagtggtggcctaactacggctacactagaagaacagtatttggtatctgcgctctgctgaagccagttaccttcggaaaaagagttggtagctcttgatccggcaaacaaaccaccgctggtagcggtggtttttttgtttgcaagcagcagattacgcgcagaaaaaaaggatctcaagaagatcctttgatcttttctacggggtctgacgctcagtggaacgaaaactcacgttaagggattttggtcatgagattatcaaaaaggatcttcacctagatccttttaaattaaaaatgaagttttaaatcaatctaaagtatatatgagtaaacttggtctgacagttaccaatgcttaatcagtgaggcacctatctcagcgatctgtctatttcgttcatccatagttgcctgactccccgtcgtgtagataactacgatacgggagggcttaccatctggccccagtgctgcaatgataccgcgagacccacgctcaccggctccagatttatcagcaataaaccagccagccggaagggccgagcgcagaagtggtcctgcaactttatccgcctccatccagtctattaattgttgccgggaagctagagtaagtagttcgccagttaatagtttgcgcaacgttgttgccattgctacaggcatcgtggtgtcacgctcgtcgtttggtatggcttcattcagctccggttcccaacgatcaaggcgagttacatgatcccccatgttgtgcaaaaaagcggttagctccttcggtcctccgatcgttgtcagaagtaagttggccgcagtgttatcactcatggttatggcagcactgcataattctcttactgtcatgccatccgtaagatgcttttctgtgactggtgagtactcaaccaagtcattctgagaatagtgtatgcggcgaccgagttgctcttgcccggcgtcaatacgggataataccgcgccacatagcagaactttaaaagtgctcatcattggaaaacgttcttcggggcgaaaactctcaaggatcttaccgctgttgagatccagttcgatgtaacccactcgtgcacccaactgatcttcagcatcttttactttcaccagcgtttctgggtgagcaaaaacaggaaggcaaaatgccgcaaaaaagggaataagggcgacacggaaatgttgaatactcatactcttcctttttcaatattattgaagcatttatcagggttattgtctcatgagcggatacatatttgaatgtatttagaaaaataaacaaataggggttccgcgcacatttccccgaaaagtgccacctgacgtcgacggatcgggagatcaacttgtttattgcagcttataatggttacaaataaagcaatagcatcacaaatttcacaaataaagcatttttttcactgcattctagttgtggtttgtccaaactcatcaatgtatcttatcatgtctggatcaactggataactcaagctaaccaaaatcatcccaaacttcccaccccataccctattaccactgccaattacctgtggtttcatttactctaaacctgtgattcctctgaattattttcattttaaagaaattgtatttgttaaatatgtactacaaacttagtagt